European Patent Application EP 4 190 817 A1, published June 7, 2023. Title: ANTI-MUC16 ANTIBODIES AND USES THEREOF. Applicant: MEMORIAL SLOAN-KETTERING CANCER CENTER. The sequence listing filed with the application follows.

SEQUENCE LISTING (175 sequences)

SEQ ID NO: 1 - protein, 122 aa, synthetic construct
  REGION 1..122: note = 10C6 VH
QVTLKESGPGILQPSQTLSLTCSFSGFSLNTLGMGVGWIRQPSGKGLEWLAHIWWDDDKYYNPALKSRLTISKDSSKNQVFLKIANVDTADIATYYCSRIGTAQATDALDYWGQGTSVTVSS

SEQ ID NO: 2 - protein, 109 aa, synthetic construct
  REGION 1..109: note = 10C6 VL
DIVLTQSPASLAVSLGQRATISYRASKSVSTSGYSYMHWNQQKPGQPPRLLIYLVSNLESGVPARFSGSGSGTDFTLNIHPVEEEDAATYYCQHIRELTRSEGGPSWKN

SEQ ID NO: 3 - protein, 7 aa, synthetic construct
  REGION 1..7: note = 10C6 HCDR1 (KABAT)
TLGMGVG

SEQ ID NO: 4 - protein, 16 aa, synthetic construct
  REGION 1..16: note = 10C6 HCDR2 (KABAT)
HIWWDDDKYYNPALKS

SEQ ID NO: 5 - protein, 12 aa, synthetic construct
  REGION 1..12: note = 10C6 HCDR3 (KABAT)
IGTAQATDALDY

SEQ ID NO: 6 - protein, 15 aa, synthetic construct
  REGION 1..15: note = 10C6 LCDR1 (KABAT)
RASKSVSTSGYSYMH

SEQ ID NO: 7 - protein, 7 aa, synthetic construct
  REGION 1..7: note = 10C6 LCDR2 (KABAT)
LVSNLES

SEQ ID NO: 8 - protein, 9 aa, synthetic construct
  REGION 1..9: note = 10C6 LCDR3 (KABAT)
QHIRELTRS

SEQ ID NO: 9 - protein, 9 aa, synthetic construct
  REGION 1..9: note = 10C6 HCDR1 (CHOTHIA)
GFSLNTLGM

SEQ ID NO: 10 - skipped

SEQ ID NO: 11 - protein, 10 aa, synthetic construct
  REGION 1..10: note = 10C6 HCDR3 (CHOTHIA)
GTAQATDALD

SEQ ID NO: 12 - protein, 11 aa, synthetic construct
  REGION 1..11: note = 10C6 LCDR1 (CHOTHIA)
SKSVSTSGYSY

SEQ ID NO: 13 - skipped

SEQ ID NO: 14 - protein, 6 aa, synthetic construct
  REGION 1..6: note = 10C6 LCDR3 (CHOTHIA)
IRELTR

SEQ ID NO: 15 - protein, 10 aa, synthetic construct
  REGION 1..10: note = 10C6 HCDR1 (IMGT)
GFSLNTLGMG

SEQ ID NO: 16 - protein, 7 aa, synthetic construct
  REGION 1..7: note = 10C6 HCDR2 (IMGT)
IWWDDDK

SEQ ID NO: 17 - protein, 14 aa, synthetic construct
  REGION 1..14: note = 10C6 HCDR3 (IMGT)
SRIGTAQATDALDY

SEQ ID NO: 18 - protein, 10 aa, synthetic construct
  REGION 1..10: note = 10C6 LCDR1 (IMGT)
KSVSTSGYSY

SEQ ID NO: 19 - skipped

SEQ ID NO: 20 - protein, 9 aa, synthetic construct
  REGION 1..9: note = 10C6 LCDR3 (IMGT)
QHIRELTRS

SEQ ID NO: 21 - protein, 123 aa, synthetic construct
  REGION 1..123: note = 7B12 VH
QVTLKESGPGILQPSQTLSLTCSFSGFSLSTVGMGVGWSRQPSGKGLEWLAHIWWDDEDKYYNPALKSRLTISKDTSKNQVFLKIANVDTADSATYYCTRIGTAQATDALDYWGQGTSVTVSS

SEQ ID NO: 22 - protein, 112 aa, synthetic construct
  REGION 1..112: note = 7B12 VL
DIVMTQAAPSVSVTPGESVSISCRSSKSLRKSNGNTYLYWFLQRPGQSPQRLIYYMSNLASGVPDRFSGRGSGTDFTLRISRVEAEDVGVYYCMQSLEYPLTFGGGTKLKIK

SEQ ID NO: 23 - protein, 7 aa, synthetic construct
  REGION 1..7: note = 7B12 HCDR1 (KABAT)
TVGMGVG

SEQ ID NO: 24 - protein, 17 aa, synthetic construct
  REGION 1..17: note = 7B12 HCDR2 (KABAT)
HIWWDDEDKYYNPALKS

SEQ ID NO: 25 - protein, 12 aa, synthetic construct
  REGION 1..12: note = 7B12 HCDR3 (KABAT)
IGTAQATDALDY

SEQ ID NO: 26 - protein, 16 aa, synthetic construct
  REGION 1..16: note = 7B12 LCDR1 (KABAT)
RSSKSLRKSNGNTYLY

SEQ ID NO: 27 - protein, 7 aa, synthetic construct
  REGION 1..7: note = 7B12 LCDR2 (KABAT)
YMSNLAS

SEQ ID NO: 28 - protein, 9 aa, synthetic construct
  REGION 1..9: note = 7B12 LCDR3 (KABAT)
MQSLEYPLT

SEQ ID NO: 29 - protein, 9 aa, synthetic construct
  REGION 1..9: note = 7B12 HCDR1 (CHOTHIA)
GFSLSTVGM

SEQ ID NO: 30 - protein, 4 aa, synthetic construct
  REGION 1..4: note = 7B12 HCDR2 (CHOTHIA)
WDDE

SEQ ID NO: 31 - protein, 10 aa, synthetic construct
  REGION 1..10: note = 7B12 HCDR3 (CHOTHIA)
GTAQATDALD

SEQ ID NO: 32 - protein, 12 aa, synthetic construct
  REGION 1..12: note = 7B12 LCDR1 (CHOTHIA)
SKSLRKSNGNTY

SEQ ID NO: 33 - skipped

SEQ ID NO: 34 - protein, 6 aa, synthetic construct
  REGION 1..6: note = 7B12 LCDR3 (CHOTHIA)
SLEYPL

SEQ ID NO: 35 - protein, 10 aa, synthetic construct
  REGION 1..10: note = 7B12 HCDR1 (IMGT)
GFSLSTVGMG

SEQ ID NO: 36 - protein, 8 aa, synthetic construct
  REGION 1..8: note = 7B12 HCDR2 (IMGT)
IWWDDEDK

SEQ ID NO: 37 - protein, 14 aa, synthetic construct
  REGION 1..14: note = 7B12 HCDR3 (IMGT)
TRIGTAQATDALDY

SEQ ID NO: 38 - protein, 11 aa, synthetic construct
  REGION 1..11: note = 7B12 LCDR1 (IMGT)
KSLRKSNGNTY

SEQ ID NO: 39 - skipped

SEQ ID NO: 40 - protein, 9 aa, synthetic construct
  REGION 1..9: note = 7B12 LCDR3 (IMGT)
MQSLEYPLT

SEQ ID NO: 41 - protein, 122 aa, synthetic construct
  REGION 1..122: note = 19C11 VH
QVNLKESGPGKLQPSQTLSLTCSFSGFSLSTLGMGVGWIRQSSGKGLEWLAHIWWDDDKYYNPALKSRLTISRATSKNQVFLKIVNVGTADTATYYCARIGTAQATDALDYWGQGTSVTVSS

SEQ ID NO: 42 - protein, 112 aa, synthetic construct
  REGION 1..112: note = 19C11 VL
DIVMTQAAPSIPVTPGESVSISCRSSKSLLHSNGNTYLYWFLQRPGQSPQRLIYYMSNLASGVPDRFSGRGSGTDFTLKISRVEAGDVGVYYCMQGLEHPLTFGGGTKLEIK

SEQ ID NO: 43 - protein, 7 aa, synthetic construct
  REGION 1..7: note = 19C11 HCDR1 (KABAT)
TLGMGVG

SEQ ID NO: 44 - protein, 16 aa, synthetic construct
  REGION 1..16: note = 19C11 HCDR2 (KABAT)
HIWWDDDKYYNPALKS

SEQ ID NO: 45 - protein, 12 aa, synthetic construct
  REGION 1..12: note = 19C11 HCDR3 (KABAT)
IGTAQATDALDY

SEQ ID NO: 46 - protein, 16 aa, synthetic construct
  REGION 1..16: note = 19C11 LCDR1 (KABAT)
RSSKSLLHSNGNTYLY

SEQ ID NO: 47 - protein, 7 aa, synthetic construct
  REGION 1..7: note = 19C11 LCDR2 (KABAT)
YMSNLAS

SEQ ID NO: 48 - protein, 9 aa, synthetic construct
  REGION 1..9: note = 19C11 LCDR3 (KABAT)
MQGLEHPLT

SEQ ID NO: 49 - protein, 9 aa, synthetic construct
  REGION 1..9: note = 19C11 HCDR1 (CHOTHIA)
GFSLSTLGM

SEQ ID NO: 50 - skipped

SEQ ID NO: 51 - protein, 10 aa, synthetic construct
  REGION 1..10: note = 19C11 HCDR3 (CHOTHIA)
GTAQATDALD

SEQ ID NO: 52 - protein, 12 aa, synthetic construct
  REGION 1..12: note = 19C11 LCDR1 (CHOTHIA)
SKSLLHSNGNTY

SEQ ID NO: 53 - skipped

SEQ ID NO: 54 - protein, 6 aa, synthetic construct
  REGION 1..6: note = 19C11 LCDR3 (CHOTHIA)
GLEHPL

SEQ ID NO: 55 - protein, 10 aa, synthetic construct
  REGION 1..10: note = 19C11 HCDR1 (IMGT)
GFSLSTLGMG

SEQ ID NO: 56 - protein, 7 aa, synthetic construct
  REGION 1..7: note = 19C11 HCDR2 (IMGT)
IWWDDDK

SEQ ID NO: 57 - protein, 14 aa, synthetic construct
  REGION 1..14: note = 19C11 HCDR3 (IMGT)
ARIGTAQATDALDY

SEQ ID NO: 58 - protein, 11 aa, synthetic construct
  REGION 1..11: note = 19C11 LCDR1 (IMGT)
KSLLHSNGNTY

SEQ ID NO: 59 - skipped

SEQ ID NO: 60 - protein, 9 aa, synthetic construct
  REGION 1..9: note = 19C11 LCDR3 (IMGT)
MQGLEHPLT

SEQ ID NO: 61 - protein, 122 aa, synthetic construct
  REGION 1..122: note = 16C5 VH
QVTLKESGPGILQPSQTLSLTCSFSGFSLNTLGMGVGWIRQPSGKGLEWLAHIWWDDDKYYYPALKSRLTISRDTSKNQVFLKIANVDTADTATYYCARIGTAQATDALDYWGQGTSVTVSS

SEQ ID NO: 62 - protein, 109 aa, synthetic construct
  REGION 1..109: note = 16C5 VL
ELDMTQTPPSLSASVGETVRIRCLASEDIYSGISWYQQKPGKPPTLLIYGASNLESGVPPRFSGSGSGTDYTLTIGGVQAEDAATYYCLGGYSYSSTLTFGAGTNVEIK

SEQ ID NO: 63 - protein, 7 aa, synthetic construct
  REGION 1..7: note = 16C5 HCDR1 (KABAT)
TLGMGVG

SEQ ID NO: 64 - protein, 16 aa, synthetic construct
  REGION 1..16: note = 16C5 HCDR2 (KABAT)
HIWWDDDKYYYPALKS

SEQ ID NO: 65 - protein, 12 aa, synthetic construct
  REGION 1..12: note = 16C5 HCDR3 (KABAT)
IGTAQATDALDY

SEQ ID NO: 66 - protein, 11 aa, synthetic construct
  REGION 1..11: note = 16C5 LCDR1 (KABAT)
LASEDIYSGIS

SEQ ID NO: 67 - protein, 7 aa, synthetic construct
  REGION 1..7: note = 16C5 LCDR2 (KABAT)
GASNLES

SEQ ID NO: 68 - protein, 11 aa, synthetic construct
  REGION 1..11: note = 16C5 LCDR3 (KABAT)
LGGYSYSSTLT

SEQ ID NO: 69 - protein, 9 aa, synthetic construct
  REGION 1..9: note = 16C5 HCDR1 (CHOTHIA)
GFSLNTLGM

SEQ ID NO: 70 - skipped

SEQ ID NO: 71 - protein, 10 aa, synthetic construct
  REGION 1..10: note = 16C5 HCDR3 (CHOTHIA)
GTAQATDALD

SEQ ID NO: 72 - protein, 7 aa, synthetic construct
  REGION 1..7: note = 16C5 LCDR1 (CHOTHIA)
SEDIYSG

SEQ ID NO: 73 - skipped

SEQ ID NO: 74 - protein, 8 aa, synthetic construct
  REGION 1..8: note = 16C5 LCDR3 (CHOTHIA)
GYSYSSTL

SEQ ID NO: 75 - protein, 10 aa, synthetic construct
  REGION 1..10: note = 16C5 HCDR1 (IMGT)
GFSLNTLGMG

SEQ ID NO: 76 - protein, 7 aa, synthetic construct
  REGION 1..7: note = 16C5 HCDR2 (IMGT)
IWWDDDK

SEQ ID NO: 77 - protein, 14 aa, synthetic construct
  REGION 1..14: note = 16C5 HCDR3 (IMGT)
ARIGTAQATDALDY

SEQ ID NO: 78 - protein, 6 aa, synthetic construct
  REGION 1..6: note = 16C5 LCDR1 (IMGT)
EDIYSG

SEQ ID NO: 79 - skipped

SEQ ID NO: 80 - protein, 11 aa, synthetic construct
  REGION 1..11: note = 16C5 LCDR3 (IMGT)
LGGYSYSSTLT

SEQ ID NO: 81 - protein, 123 aa, synthetic construct
  REGION 1..123: note = 18C6 VH
QVTLKESGPGILQPSQTLSLTCSFSGFSLSTVGMGVGWSRQPSGKGLEWLAHIWWDDEDKYYNPALKSRLTISKDTSKNQVFLKIANVDTADTATYYCTRIGTAQATDALDYWGQGTSVTVSS

SEQ ID NO: 82 - protein, 112 aa, synthetic construct
  REGION 1..112: note = 18C6 VL
DIVMTQAAPSVPVTPGESVSISCRSSKSLLHSNGNTYLYWFLQRPGQSPQRLIYYMSNLASGVPDRFSGRGSGTDFTLRISRVEAEDVGVYYCMQSLEYPLTFGGGTKLEIK

SEQ ID NO: 83 - protein, 7 aa, synthetic construct
  REGION 1..7: note = 18C6 HCDR1 (KABAT)
TVGMGVG

SEQ ID NO: 84 - protein, 17 aa, synthetic construct
  REGION 1..17: note = 18C6 HCDR2 (KABAT)
HIWWDDEDKYYNPALKS

SEQ ID NO: 85 - protein, 12 aa, synthetic construct
  REGION 1..12: note = 18C6 HCDR3 (KABAT)
IGTAQATDALDY

SEQ ID NO: 86 - protein, 16 aa, synthetic construct
  REGION 1..16: note = 18C6 LCDR1 (KABAT)
RSSKSLLHSNGNTYLY

SEQ ID NO: 87 - protein, 7 aa, synthetic construct
  REGION 1..7: note = 18C6 LCDR2 (KABAT)
YMSNLAS

SEQ ID NO: 88 - protein, 9 aa, synthetic construct
  REGION 1..9: note = 18C6 LCDR3 (KABAT)
MQSLEYPLT

SEQ ID NO: 89 - protein, 9 aa, synthetic construct
  REGION 1..9: note = 18C6 HCDR1 (CHOTHIA)
GFSLSTVGM

SEQ ID NO: 90 - protein, 4 aa, synthetic construct
  REGION 1..4: note = 18C6 HCDR2 (CHOTHIA)
WDDE

SEQ ID NO: 91 - protein, 10 aa, synthetic construct
  REGION 1..10: note = 18C6 HCDR3 (CHOTHIA)
GTAQATDALD

SEQ ID NO: 92 - protein, 12 aa, synthetic construct
  REGION 1..12: note = 18C6 LCDR1 (CHOTHIA)
SKSLLHSNGNTY

SEQ ID NO: 93 - skipped

SEQ ID NO: 94 - protein, 6 aa, synthetic construct
  REGION 1..6: note = 18C6 LCDR3 (CHOTHIA)
SLEYPL

SEQ ID NO: 95 - protein, 10 aa, synthetic construct
  REGION 1..10: note = 18C6 HCDR1 (IMGT)
GFSLSTVGMG

SEQ ID NO: 96 - protein, 8 aa, synthetic construct
  REGION 1..8: note = 18C6 HCDR2 (IMGT)
IWWDDEDK

SEQ ID NO: 97 - protein, 14 aa, synthetic construct
  REGION 1..14: note = 18C6 HCDR3 (IMGT)
TRIGTAQATDALDY

SEQ ID NO: 98 - protein, 11 aa, synthetic construct
  REGION 1..11: note = 18C6 LCDR1 (IMGT)
KSLLHSNGNTY

SEQ ID NO: 99 - skipped

SEQ ID NO: 100 - protein, 9 aa, synthetic construct
  REGION 1..9: note = 18C6 LCDR3 (IMGT)
MQSLEYPLT

SEQ ID NO: 101 - protein, 123 aa, synthetic construct
  REGION 1..123: note = 10C6-18C6 VH consensus
  VARIANT 3: note = Xaa = Thr or Asn
  VARIANT 11: note = Xaa = Ile or Lys
  VARIANT 30: note = Xaa = Asn or Ser
  VARIANT 32: note = Xaa = Val or Leu
  VARIANT 39: note = Xaa = Ser or Ile
  VARIANT 42: note = Xaa = Pro or Ser
  VARIANT 58: note = Xaa = Glu or absent
  VARIANT 63: note = Xaa = Asn or Tyr
  VARIANT 74: note = Xaa = Lys or Arg
  VARIANT 75: note = Xaa = Ala or Asp
  VARIANT 76: note = Xaa = Thr or Ser
  VARIANT 86: note = Xaa = Val or Ala
  VARIANT 89: note = Xaa = Gly or Asp
  VARIANT 93: note = Xaa = Thr, Ile or Ser
  VARIANT 99: note = Xaa = Thr, Ser or Ala
QVXLKESGPGXLQPSQTLSLTCSFSGFSLXTXGMGVGWXRQXSGKGLEWLAHIWWDDXDKYYXPALKSRLTISXXXSKNQVFLKIXNVXTADXATYYCXRIGTAQATDALDYWGQGTSVTVSS

SEQ ID NO: 102 - protein, 112 aa, synthetic construct
  REGION 1..112: note = 7B12, 19C11, 18C6 VL consensus
  VARIANT 11: note = Xaa = Ile or Val
  VARIANT 12: note = Xaa = Pro or Ser
  VARIANT 30: note = Xaa = Arg or Leu
  VARIANT 31: note = Xaa = Lys or His
  VARIANT 79: note = Xaa = Arg or Lys
  VARIANT 86: note = Xaa = Glu or Gly
  VARIANT 96: note = Xaa = Ser or Gly
  VARIANT 99: note = Xaa = Tyr or His
DIVMTQAAPSXXVTPGESVSISCRSSKSLXXSNGNTYLYWFLQRPGQSPQRLIYYMSNLASGVPDRFSGRGSGTDFTLXISRVEAXDVGVYYCMQXLEXPLTFGGGTKLEIK

SEQ ID NO: 103 - protein, 7 aa, synthetic construct
  REGION 1..7: note = HCDR1 KABAT CONSENSUS
  VARIANT 2: note = Xaa = Lue or Val
TXGMGVG

SEQ ID NO: 104 - protein, 17 aa, synthetic construct
  REGION 1..17: note = HCDR2 KABAT CONSENSUS
  VARIANT 7: note = Xaa = Glu or Absent
  VARIANT 12: note = Xaa = Tyr or Asn
HIWWDDXDKYYXPALKS

SEQ ID NO: 105 - protein, 12 aa, synthetic construct
  REGION 1..12: note = HCDR3 KABAT CONSENSUS
IGTAQATDALDY

SEQ ID NO: 106 - protein, 16 aa, synthetic construct
  REGION 1..16: note = 7B12, 19C11, 18C6 LCDR2 KABAT CONSENSUS
  VARIANT 7: note = Xaa = Arg or Leu
  VARIANT 8: note = Xaa = Lys or His
RSSKSLXXSNGNTYLY

SEQ ID NO: 107 - protein, 7 aa, synthetic construct
  REGION 1..7: note = 7B12, 19C11, 18C6 LCDR2 KABAT CONSENSUS
YMSNLAS

SEQ ID NO: 108 - protein, 9 aa, synthetic construct
  REGION 1..9: note = 7B12, 19C11, 18C6 LCDR3 KABAT CONSENSUS
  VARIANT 3: note = Xaa = Gly or Ser
  VARIANT 6: note = Xaa = His or Tyr
MQXLEXPLT

SEQ ID NO: 109 - protein, 9 aa, synthetic construct
  REGION 1..9: note = 10C6-18C6 HCDR1 CHOTHIA CONSENSUS
  VARIANT 5: note = Xaa = Asn or Ser
  VARIANT 7: note = Xaa = Leu or Val
GFSLXTXGM

SEQ ID NO: 110 - skipped

SEQ ID NO: 111 - protein, 10 aa, synthetic construct
  REGION 1..10: note = 10C6-18C6 HCDR3 CHOTHIA CONSENSUS
GTAQATDALD

SEQ ID NO: 112 - protein, 12 aa, synthetic construct
  REGION 1..12: note = 7B12, 19C11, 18C6 LCDR1 CHOTHIA CONSENSUS
  VARIANT 5: note = Xaa = Leu or Arg
  VARIANT 6: note = Xaa = His or Lys
SKSLXXSNGNTY

SEQ ID NO: 113 - skipped

SEQ ID NO: 114 - protein, 6 aa, synthetic construct
  REGION 1..6: note = 7B12, 19C11, 18C6 LCDR3 CHOTHIA CONSENSUS
  VARIANT 1: note = Xaa = Gly or Ser
  VARIANT 4: note = Xaa = His or Tyr
XLEXPL

SEQ ID NO: 115 - protein, 10 aa, synthetic construct
  REGION 1..10: note = 10C6-18C6 HCDR1 IMGT CONSENSUS
  VARIANT 5: note = Xaa = Asn or Ser
  VARIANT 7: note = Xaa = Val or Leu
GFSLXTXGMG

SEQ ID NO: 116 - protein, 8 aa, synthetic construct
  REGION 1..8: note = 10C6-18C6 HCDR2 IMGT CONSENSUS
  VARIANT 6: note = Xaa = Glu or Absent
IWWDDXDK

SEQ ID NO: 117 - protein, 14 aa, synthetic construct
  REGION 1..14: note = 10C6-18C6 HCDR3 IMGT CONSENSUS
  VARIANT 1: note = Xaa = Thr, Ala or Ser
XRIGTAQATDALDY

SEQ ID NO: 118 - protein, 11 aa, synthetic construct
  REGION 1..11: note = 7B12, 19C11, 18C6 LCDR1 IMGT CONSENSUS
  VARIANT 4: note = Xaa = Val or Leu
  VARIANT 5: note = Xaa = His or Lys
KSLXXSNGNTY

SEQ ID NO: 119 - skipped

SEQ ID NO: 120 - protein, 9 aa, synthetic construct
  REGION 1..9: note = 7B12, 19C11, 18C6 LCDR3 IMGT CONSENSUS
MQSLEYPLT

SEQ ID NO: 121 - protein, 42 aa, synthetic construct
  REGION 1..42: note = MUC16c114 F primer
CCATGCGATATCGCCACCATGGTGAACTTCTCGCCACTGGCT

SEQ ID NO: 122 - protein, 34 aa, synthetic construct
  REGION 1..34: note = MUC16c114 R primer
TACGGCGGCCGCTTGCAGATCCTCCAGGTCTAGG

SEQ ID NO: 123 - protein, 45 aa, synthetic construct
  REGION 1..45: note = MUC16c344 F primer
CCATGCGATATCGCCACCATGGTGACAGGCCCTGGGCTGGACAGA

SEQ ID NO: 124 - protein, 34 aa, synthetic construct; identical to SEQ ID NO: 122
  REGION 1..34: note = MUC16c344 R primer

SEQ ID NO: 125 - protein, 31 aa, synthetic construct
  REGION 1..31: note = MUC16c57-114 F primer
CCATGCGATATCAAACTTCTCGCCACTGGCT

SEQ ID NO: 126 - protein, 33 aa, synthetic construct
  REGION 1..33: note = MUC16c57-114 R primer
AGATCTAACCATGGGAAGGTCAGAATTCCCAGT

SEQ ID NO: 127 - protein, 31 aa, synthetic construct
  REGION 1..31: note = 117-244LGALS3 F primer
CCATGCGATATCACCTTATAACCTGCCTTTG

SEQ ID NO: 128 - protein, 30 aa, synthetic construct
  REGION 1..30: note = 117-244LGALS3 R primer
AGATCTAACCATGGTATATGAAGCACTGGT

SEQ ID NO: 129 - protein, 55 aa, synthetic construct
  REGION 1..55: note = 55mer immunizing peptide
NFSPLARRVDRVAIYEEFLRMTRNGTQLQNFTLDRSSVLVDGYSPNRNEPLTGNS

SEQ ID NO: 130 - protein, 18 aa, synthetic construct
  REGION 1..18: note = 18mer immunizing peptide
CTRNGTQLQNFTLDRSSV

SEQ ID NO: 131 - protein, 15 aa, synthetic construct
  REGION 1..15: note = 15mer immunizing peptide
CGTQLQNFTLDRSSV

SEQ ID NO: 132 - protein, 344 aa, synthetic construct
  REGION 1..344: note = MUC16c344
WELSQLTHGVTQLGFYVLDRDSLFINGYAPQNLSIRGEYQINFHIVNQNLSNPDPTSSEYITLLRDIQDKVTTLYKGSQLHDTFRFCLVTNLTMDSVLVTVKALFSSNLDPSLVEQVFLDKTLNASFHQLGSTYQLVDIHVTEMESSVYQPTSSSSTQHFYLNFTITNLPYSQDKAQPGTTNYQRNKRNIEDALNQLFRNSSIKSYFSDCQVSTFRSVPNRHHTGVDSLCNFSPLARRVDRVAIYEEFLRMTRNGTQLQNFTLDRSSVLVDGYSPNRNEPLTGNSDLPFWAVILIGLAGLLGLITCLICGVLVTTRRRKKEGEYNVQQQCPGYYQSHLDLEDLQ

SEQ ID NO: 133 - protein, 114 aa, synthetic construct
  REGION 1..114: note = MUC16c114
NFSPLARRVDRVAIYEEFLRMTRNGTQLQNFTLDRSSVLVDGYSPNRNEPLTGNSDLPFWAVILIGLAGLLGLITCLICGVLVTTRRRKKEGEYNVQQQCPGYYQSHLDLEDLQ

SEQ ID NO: 134 - protein, 80 aa, synthetic construct
  REGION 1..80: note = MUC16c86
NFSPLARRVDRVAIYEEFLRMDLPFWAVILIGLAGLLGLITCLICGVLVTTRRRKKEGEYNVQQQCPGYYQSHLDLEDLQ

SEQ ID NO: 135 - protein, 86 aa, synthetic construct
  REGION 1..86: note = MUC16c80
NFSPLARRVDRVAIYEEFLRMTRNGTQLQNFTLDRSSVLVDGYSPNRNEPLTGNSDLPFWAVILIGLAGLLGLITCLICGDLEDLQ

SEQ ID NO: 136 - protein, 14507 aa, Homo sapiens
  REGION 1..14507: note = Immature Human MUC16 amino acid sequence (NP_078966.2)
MLKPSGLPGSSSPTRSLMTGSRSTKATPEMDSGLTGATLSPKTSTGAIVVTEHTLPFTSPDKTLASPTSSVVGRTTQSLGVMSSALPESTSRGMTHSEQRTSPSLSPQVNGTPSRNYPATSMVSGLSSPRTRTSSTEGNFTKEASTYTLTVETTSGPVTEKYTVPTETSTTEGDSTETPWDTRYIPVKITSPMKTFADSTASKENAPVSMTPAETTVTDSHTPGRTNPSFGTLYSSFLDLSPKGTPNSRGETSLELILSTTGYPFSSPEPGSAGHSRISTSAPLSSSASVLDNKISETSIFSGQSLTSPLSPGVPEARASTMPNSAIPFSMTLSNAETSAERVRSTISSLGTPSISTKQTAETILTFHAFAETMDIPSTHIAKTLASEWLGSPGTLGGTSTSALTTTSPSTTLVSEETNTHHSTSGKETEGTLNTSMTPLETSAPGEESEMTATLVPTLGFTTLDSKIRSPSQVSSSHPTRELRTTGSTSGRQSSSTAAHGSSDILRATTSSTSKASSWTSESTAQQFSEPQHTQWVETSPSMKTERPPASTSVAAPITTSVPSVVSGFTTLKTSSTKGIWLEETSADTLIGESTAGPTTHQFAVPTGISMTGGSSTRGSQGTTHLLTRATASSETSADLTLATNGVPVSVSPAVSKTAAGSSPPGGTKPSYTMVSSVIPETSSLQSSAFREGTSLGLTPLNTRHPFSSPEPDSAGHTKISTSIPLLSSASVLEDKVSATSTFSHHKATSSITTGTPEISTKTKPSSAVLSSMTLSNAATSPERVRNATSPLTHPSPSGEETAGSVLTLSTSAETTDSPNIHPTGTLTSESSESPSTLSLPSVSGVKTTFSSSTPSTHLFTSGEETEETSNPSVSQPETSVSRVRTTLASTSVPTPVFPTMDTWPTRSAQFSSSHLVSELRATSSTSVTNSTGSALPKISHLTGTATMSQTNRDTFNDSAAPQSTTWPETSPRFKTGLPSATTTVSTSATSLSATVMVSKFTSPATSSMEATSIREPSTTILTTETTNGPGSMAVASTNIPIGKGYITEGRLDTSHLPIGTTASSETSMDFTMAKESVSMSVSPSQSMDAAGSSTPGRTSQFVDTFSDDVYHLTSREITIPRDGTSSALTPQMTATHPPSPDPGSARSTWLGILSSSPSSPTPKVTMSSTFSTQRVTTSMIMDTVETSRWNMPNLPSTTSLTPSNIPTSGAIGKSTLVPLDTPSPATSLEASEGGLPTLSTYPESTNTPSIHLGAHASSESPSTIKLTMASVVKPGSYTPLTFPSIETHIHVSTARMAYSSGSSPEMTAPGETNTGSTWDPTTYITTTDPKDTSSAQVSTPHSVRTLRTTENHPKTESATPAAYSGSPKISSSPNLTSPATKAWTITDTTEHSTQLHYTKLAEKSSGFETQSAPGPVSVVIPTSPTIGSSTLELTSDVPGEPLVLAPSEQTTITLPMATWLSTSLTEEMASTDLDISSPSSPMSTFAIFPPMSTPSHELSKSEADTSAIRNTDSTTLDQHLGIRSLGRTGDLTTVPITPLTTTWTSVIEHSTQAQDTLSATMSPTHVTQSLKDQTSIPASASPSHLTEVYPELGTQGRSSSEATTFWKPSTDTLSREIETGPTNIQSTPPMDNTTTGSSSSGVTLGIAHLPIGTSSPAETSTNMALERRSSTATVSMAGTMGLLVTSAPGRSISQSLGRVSSVLSESTTEGVTDSSKGSSPRLNTQGNTALSSSLEPSYAEGSQMSTSIPLTSSPTTPDVEFIGGSTFWTKEVTTVMTSDISKSSARTESSSATLMSTALGSTENTGKEKLRTASMDLPSPTPSMEVTPWISLTLSNAPNTTDSLDLSHGVHTSSAGTLATDRSLNTGVTRASRLENGSDTSSKSLSMGNSTHTSMTYTEKSEVSSSIHPRPETSAPGAETTLTSTPGNRAISLTLPFSSIPVEEVISTGITSGPDINSAPMTHSPITPPTIVWTSTGTIEQSTQPLHAVSSEKVSVQTQSTPYVNSVAVSASPTHENSVSSGSSTSSPYSSASLESLDSTISRRNAITSWLWDLTTSLPTTTWPSTSLSEALSSGHSGVSNPSSTTTEFPLFSAASTSAAKQRNPETETHGPQNTAASTLNTDASSVTGLSETPVGASISSEVPLPMAITSRSDVSGLTSESTANPSLGTASSAGTKLTRTISLPTSESLVSFRMNKDPWTVSIPLGSHPTTNTETSIPVNSAGPPGLSTVASDVIDTPSDGAESIPTVSFSPSPDTEVTTISHFPEKTTHSFRTISSLTHELTSRVTPIPGDWMSSAMSTKPTGASPSITLGERRTITSAAPTTSPIVLTASFTETSTVSLDNETTVKTSDILDARKTNELPSDSSSSSDLINTSIASSTMDVTKTASISPTSISGMTASSSPSLFSSDRPQVPTSTTETNTATSPSVSSNTYSLDGGSNVGGTPSTLPPFTITHPVETSSALLAWSRPVRTFSTMVSTDTASGENPTSSNSVVTSVPAPGTWTSVGSTTDLPAMGFLKTSPAGEAHSLLASTIEPATAFTPHLSAAVVTGSSATSEASLLTTSESKAIHSSPQTPTTPTSGANWETSATPESLLVVTETSDTTLTSKILVTDTILFSTVSTPPSKFPSTGTLSGASFPTLLPDTPAIPLTATEPTSSLATSFDSTPLVTIASDSLGTVPETTLTMSETSNGDALVLKTVSNPDRSIPGITIQGVTESPLHPSSTSPSKIVAPRNTTYEGSITVALSTLPAGTTGSLVFSQSSENSETTALVDSSAGLERASVMPLTTGSQGMASSGGIRSGSTHSTGTKTFSSLPLTMNPGEVTAMSEITTNRLTATQSTAPKGIPVKPTSAESGLLTPVSASSSPSKAFASLTTAPPTWGIPQSTLTFEFSEVPSLDTKSASLPTPGQSLNTIPDSDASTASSSLSKSPEKNPRARMMTSTKAISASSFQSTGFTETPEGSASPSMAGHEPRVPTSGTGDPRYASESMSYPDPSKASSAMTSTSLASKLTTLFSTGQAARSGSSSSPISLSTEKETSFLSPTASTSRKTSLFLGPSMARQPNILVHLQTSALTLSPTSTLNMSQEEPPELTSSQTIAEEEGTTAETQTLTFTPSETPTSLLPVSSPTEPTARRKSSPETWASSISVPAKTSLVETTDGTLVTTIKMSSQAAQGNSTWPAPAEETGSSPAGTSPGSPEMSTTLKIMSSKEPSISPEIRSTVRNSPWKTPETTVPMETTVEPVTLQSTALGSGSTSISHLPTGTTSPTKSPTENMLATERVSLSPSPPEAWTNLYSGTPGGTRQSLATMSSVSLESPTARSITGTGQQSSPELVSKTTGMEFSMWHGSTGGTTGDTHVSLSTSSNILEDPVTSPNSVSSLTDKSKHKTETWVSTTAIPSTVLNNKIMAAEQQTSRSVDEAYSSTSSWSDQTSGSDITLGASPDVTNTLYITSTAQTTSLVSLPSGDQGITSLTNPSGGKTSSASSVTSPSIGLETLRANVSAVKSDIAPTAGHLSQTSSPAEVSILDVTTAPTPGISTTITTMGTNSISTTTPNPEVGMSTMDSTPATERRTTSTEHPSTWSSTAASDSWTVTDMTSNLKVARSPGTISTMHTTSFLASSTELDSMSTPHGRITVIGTSLVTPSSDASAVKTETSTSERTLSPSDTTASTPISTFSRVQRMSISVPDILSTSWTPSSTEAEDVPVSMVSTDHASTKTDPNTPLSTFLFDSLSTLDWDTGRSLSSATATTSAPQGATTPQELTLETMISPATSQLPFSIGHITSAVTPAAMARSSGVTFSRPDPTSKKAEQTSTQLPTTTSAHPGQVPRSAATTLDVIPHTAKTPDATFQRQGQTALTTEARATSDSWNEKEKSTPSAPWITEMMNSVSEDTIKEVTSSSSVLRTLNTLDINLESGTTSSPSWKSSPYERIAPSESTTDKEAIHPSTNTVETTGWVTSSEHASHSTIPAHSASSKLTSPVVTTSTREQAIVSMSTTTWPESTRARTEPNSFLTIELRDVSPYMDTSSTTQTSIISSPGSTAITKGPRTEITSSKRISSSFLAQSMRSSDSPSEAITRLSNFPAMTESGGMILAMQTSPPGATSLSAPTLDTSATASWTGTPLATTQRFTYSEKTTLFSKGPEDTSQPSPPSVEETSSSSSLVPIHATTSPSNILLTSQGHSPSSTPPVTSVFLSETSGLGKTTDMSRISLEPGTSLPPNLSSTAGEALSTYEASRDTKAIHHSADTAVTNMEATSSEYSPIPGHTKPSKATSPLVTSHIMGDITSSTSVFGSSETTEIETVSSVNQGLQERSTSQVASSATETSTVITHVSSGDATTHVTKTQATFSSGTSISSPHQFITSTNTFTDVSTNPSTSLIMTESSGVTITTQTGPTGAATQGPYLLDTSTMPYLTETPLAVTPDFMQSEKTTLISKGPKDVSWTSPPSVAETSYPSSLTPFLVTTIPPATSTLQGQHTSSPVSATSVLTSGLVKTTDMLNTSMEPVTNSPQNLNNPSNEILATLAATTDIETIHPSINKAVTNMGTASSAHVLHSTLPVSSEPSTATSPMVPASSMGDALASISIPGSETTDIEGEPTSSLTAGRKENSTLQEMNSTTESNIILSNVSVGAITEATKMEVPSFDATFIPTPAQSTKFPDIFSVASSRLSNSPPMTISTHMTTTQTGSSGATSKIPLALDTSTLETSAGTPSVVTEGFAHSKITTAMNNDVKDVSQTNPPFQDEASSPSSQAPVLVTTLPSSVAFTPQWHSTSSPVSMSSVLTSSLVKTAGKVDTSLETVTSSPQSMSNTLDDISVTSAATTDIETTHPSINTVVTNVGTTGSAFESHSTVSAYPEPSKVTSPNVTTSTMEDTTISRSIPKSSKTTRTETETTSSLTPKLRETSISQEITSSTETSTVPYKELTGATTEVSRTDVTSSSSTSFPGPDQSTVSLDISTETNTRLSTSPIMTESAEITITTQTGPHGATSQDTFTMDPSNTTPQAGIHSAMTHGFSQLDVTTLMSRIPQDVSWTSPPSVDKTSSPSSFLSSPAMTTPSLISSTLPEDKLSSPMTSLLTSGLVKITDILRTRLEPVTSSLPNFSSTSDKILATSKDSKDTKEIFPSINTEETNVKANNSGHESHSPALADSETPKATTQMVITTTVGDPAPSTSMPVHGSSETTNIKREPTYFLTPRLRETSTSQESSFPTDTSFLLSKVPTGTITEVSSTGVNSSSKISTPDHDKSTVPPDTFTGEIPRVFTSSIKTKSAEMTITTQASPPESASHSTLPLDTSTTLSQGGTHSTVTQGFPYSEVTTLMGMGPGNVSWMTTPPVEETSSVSSLMSSPAMTSPSPVSSTSPQSIPSSPLPVTALPTSVLVTTTDVLGTTSPESVTSSPPNLSSITHERPATYKDTAHTEAAMHHSTNTAVTNVGTSGSGHKSQSSVLADSETSKATPLMSTTSTLGDTSVSTSTPNISQTNQIQTEPTASLSPRLRESSTSEKTSSTTETNTAFSYVPTGAITQASRTEISSSRTSISDLDRPTIAPDISTGMITRLFTSPIMTKSAEMTVTTQTTTPGATSQGILPWDTSTTLFQGGTHSTVSQGFPHSEITTLRSRTPGDVSWMTTPPVEETSSGFSLMSPSMTSPSPVSSTSPESIPSSPLPVTALLTSVLVTTTNVLGTTSPEPVTSSPPNLSSPTQERLTTYKDTAHTEAMHASMHTNTAVANVGTSISGHESQSSVPADSHTSKATSPMGITFAMGDTSVSTSTPAFFETRIQTESTSSLIPGLRDTRTSEEINTVTETSTVLSEVPTTTTTEVSRTEVITSSRTTISGPDHSKMSPYISTETITRLSTFPFVTGSTEMAITNQTGPIGTISQATLTLDTSSTASWEGTHSPVTQRFPHSEETTTMSRSTKGVSWQSPPSVEETSSPSSPVPLPAITSHSSLYSAVSGSSPTSALPVTSLLTSGRRKTIDMLDTHSELVTSSLPSASSFSGEILTSEASTNTETIHFSENTAETNMGTTNSMHKLHSSVSIHSQPSGHTPPKVTGSMMEDAIVSTSTPGSPETKNVDRDSTSPLTPELKEDSTALVMNSTTESNTVFSSVSLDAATEVSRAEVTYYDPTFMPASAQSTKSPDISPEASSSHSNSPPLTISTHKTIATQTGPSGVTSLGQLTLDTSTIATSAGTPSARTQDFVDSETTSVMNNDLNDVLKTSPFSAEEANSLSSQAPLLVTTSPSPVTSTLQEHSTSSLVSVTSVPTPTLAKITDMDTNLEPVTRSPQNLRNTLATSEATTDTHTMHPSINTAVANVGTTSSPNEFYFTVSPDSDPYKATSAVVITSTSGDSIVSTSMPRSSAMKKIESETTFSLIFRLRETSTSQKIGSSSDTSTVFDKAFTAATTEVSRTELTSSSRTSIQGTEKPTMSPDTSTRSVTMLSTFAGLTKSEERTIATQTGPHRATSQGTLTWDTSITTSQAGTHSAMTHGFSQLDLSTLTSRVPEYISGTSPPSVEKTSSSSSLLSLPAITSPSPVPTTLPESRPSSPVHLTSLPTSGLVKTTDMLASVASLPPNLGSTSHKIPTTSEDIKDTEKMYPSTNIAVTNVGTTTSEKESYSSVPAYSEPPKVTSPMVTSFNIRDTIVSTSMPGSSEITRIEMESTFSLAHGLKGTSTSQDPIVSTEKSAVLHKLTTGATETSRTEVASSRRTSIPGPDHSTESPDISTEVIPSLPISLGITESSNMTIITRTGPPLGSTSQGTFTLDTPTTSSRAGTHSMATQEFPHSEMTTVMNKDPEILSWTIPPSIEKTSFSSSLMPSPAMTSPPVSSTLPKTIHTTPSPMTSLLTPSLVMTTDTLGTSPEPTTSSPPNLSSTSHEILTTDEDTTAIEAMHPSTSTAATNVETTSSGHGSQSSVLADSEKTKATAPMDTTSTMGHTTVSTSMSVSSETTKIKRESTYSLTPGLRETSISQNASFSTDTSIVLSEVPTGTTAEVSRTEVTSSGRTSIPGPSQSTVLPEISTRTMTRLFASPTMTESAEMTIPTQTGPSGSTSQDTLTLDTSTTKSQAKTHSTLTQRFPHSEMTTLMSRGPGDMSWQSSPSLENPSSLPSLLSLPATTSPPPISSTLPVTISSSPLPVTSLLTSSPVTTTDMLHTSPELVTSSPPKLSHTSDERLTTGKDTTNTEAVHPSTNTAASNVEIPSSGHESPSSALADSETSKATSPMFITSTQEDTTVAISTPHFLETSRIQKESISSLSPKLRETGSSVETSSAIETSAVLSEVSIGATTEISRTEVTSSSRTSISGSAESTMLPEISTTRKIIKFPTSPILAESSEMTIKTQTSPPGSTSESTFTLDTSTTPSLVITHSTMTQRLPHSEITTLVSRGAGDVPRPSSLPVEETSPPSSQLSLSAMISPSPVSSTLPASSHSSSASVTSLLTPGQVKTTEVLDASAEPETSSPPSLSSTSVEILATSEVTTDTEKIHPFSNTAVTKVGTSSSGHESPSSVLPDSETTKATSAMGTISIMGDTSVSTLTPALSNTRKIQSEPASSLTTRLRETSTSEETSLATEANTVLSKVSTGATTEVSRTEAISFSRTSMSGPEQSTMSQDISIGTIPRISASSVLTESAKMTITTQTGPSESTLESTLNLNTATTPSWVETHSIVIQGFPHPEMTTSMGRGPGGVSWPSPPFVKETSPPSSPLSLPAVTSPHPVSTTFLAHIPPSPLPVTSLLTSGPATTTDILGTSTEPGTSSSSSLSTTSHERLTTYKDTAHTEAVHPSTNTGGTNVATTSSGYKSQSSVLADSSPMCTTSTMGDTSVLTSTPAFLETRRIQTELASSLTPGLRESSGSEGTSSGTKMSTVLSKVPTGATTEISKEDVTSIPGPAQSTISPDISTRTVSWFSTSPVMTESAEITMNTHTSPLGATTQGTSTLDTSSTTSLTMTHSTISQGFSHSQMSTLMRRGPEDVSWMSPPLLEKTRPSFSLMSSPATTSPSPVSSTLPESISSSPLPVTSLLTSGLAKTTDMLHKSSEPVTNSPANLSSTSVEILATSEVTTDTEKTHPSSNRTVTDVGTSSSGHESTSFVLADSQTSKVTSPMVITSTMEDTSVSTSTPGFFETSRIQTEPTSSLTLGLRKTSSSEGTSLATEMSTVLSGVPTGATAEVSRTEVTSSSRTSISGFAQLTVSPETSTETITRLPTSSIMTESAEMMIKTQTDPPGSTPESTHTVDISTTPNWVETHSTVTQRFSHSEMTTLVSRSPGDMLWPSQSSVEETSSASSLLSLPATTSPSPVSSTLVEDFPSASLPVTSLLNPGLVITTDRMGISREPGTSSTSNLSSTSHERLTTLEDTVDTEDMQPSTHTAVTNVRTSISGHESQSSVLSDSETPKATSPMGTTYTMGETSVSISTSDFFETSRIQIEPTSSLTSGLRETSSSERISSATEGSTVLSEVPSGATTEVSRTEVISSRGTSMSGPDQFTISPDISTEAITRLSTSPIMTESAESAITIETGSPGATSEGTLTLDTSTTTFWSGTHSTASPGFSHSEMTTLMSRTPGDVPWPSLPSVEEASSVSSSLSSPAMTSTSFFSTLPESISSSPHPVTALLTLGPVKTTDMLRTSSEPETSSPPNLSSTSAEILATSEVTKDREKIHPSSNTPVVNVGTVIYKHLSPSSVLADLVTTKPTSPMATTSTLGNTSVSTSTPAFPETMMTQPTSSLTSGLREISTSQETSSATERSASLSGMPTGATTKVSRTEALSLGRTSTPGPAQSTISPEISTETITRISTPLTTTGSAEMTITPKTGHSGASSQGTFTLDTSSRASWPGTHSAATHRSPHSGMTTPMSRGPEDVSWPSRPSVEKTSPPSSLVSLSAVTSPSPLYSTPSESSHSSPLRVTSLFTPVMMKTTDMLDTSLEPVTTSPPSMNITSDESLATSKATMETEAIQLSENTAVTQMGTISARQEFYSSYPGLPEPSKVTSPVVTSSTIKDIVSTTIPASSEITRIEMESTSTLTPTPRETSTSQEIHSATKPSTVPYKALTSATIEDSMTQVMSSSRGPSPDQSTMSQDISTEVITRLSTSPIKTESTEMTITTQTGSPGATSRGTLTLDTSTTFMSGTHSTASQGFSHSQMTALMSRTPGDVPWLSHPSVEEASSASFSLSSPVMTSSSPVSSTLPDSIHSSSLPVTSLLTSGLVKTTELLGTSSEPETSSPPNLSSTSAEILAITEVTTDTEKLEMTNVVTSGYTHESPSSVLADSVTTKATSSMGITYPTGDTNVLTSTPAFSDTSRIQTKSKLSLTPGLMETSISEETSSATEKSTVLSSVPTGATTEVSRTEAISSSRTSIPGPAQSTMSSDTSMETITRISTPLTRKESTDMAITPKTGPSGATSQGTFTLDSSSTASWPGTHSATTQRFPQSVVTTPMSRGPEDVSWPSPLSVEKNSPPSSLVSSSSVTSPSPLYSTPSGSSHSSPVPVTSLFTSIMMKATDMLDASLEPETTSAPNMNITSDESLAASKATTETEAIHVFENTAASHVETTSATEELYSSSPGFSEPTKVISPVVTSSSIRDNMVSTTMPGSSGITRIEIESMSSLTPGLRETRTSQDITSSTETSTVLYKMPSGATPEVSRTEVMPSSRTSIPGPAQSTMSLDISDEVVTRLSTSPIMTESAEITITTQTGYSLATSQVTLPLGTSMTFLSGTHSTMSQGLSHSEMTNLMSRGPESLSWTSPRFVETTRSSSSLTSLPLTTSLSPVSSTLLDSSPSSPLPVTSLILPGLVKTTEVLDTSSEPKTSSSPNLSSTSVEIPATSEIMTDTEKIHPSSNTAVAKVRTSSSVHESHSSVLADSETTITIPSMGITSAVDDTTVFTSNPAFSETRRIPTEPTFSLTPGFRETSTSEETTSITETSAVLYGVPTSATTEVSMTEIMSSNRIHIPDSDQSTMSPDIITEVITRLSSSSMMSESTQMTITTQKSSPGATAQSTLTLATTTAPLARTHSTVPPRFLHSEMTTLMSRSPENPSWKSSLFVEKTSSSSSLLSLPVTTSPSVSSTLPQSIPSSSFSVTSLLTPGMVKTTDTSTEPGTSLSPNLSGTSVEILAASEVTTDTEKIHPSSSMAVTNVGTTSSGHELYSSVSIHSEPSKATYPVGTPSSMAETSISTSMPANFETTGFEAEPFSHLTSGFRKTNMSLDTSSVTPTNTPSSPGSTHLLQSSKTDFTSSAKTSSPDWPPASQYTEIPVDIITPFNASPSITESTGITSFPESRFTMSVTESTHHLSTDLLPSAETISTGTVMPSLSEAMTSFATTGVPRAISGSGSPFSRTESGPGDATLSTIAESLPSSTPVPFSSSTFTTTDSSTIPALHEITSSSATPYRVDTSLGTESSTTEGRLVMVSTLDTSSQPGRTSSSPILDTRMTESVELGTVTSAYQVPSLSTRLTRTDGIMEHITKIPNEAAHRGTIRPVKGPQTSTSPASPKGLHTGGTKRMETTTTALKTTTTALKTTSRATLTTSVYTPTLGTLTPLNASMQMASTIPTEMMITTPYVFPDVPETTSSLATSLGAETSTALPRTTPSVFNRESETTASLVSRSGAERSPVIQTLDVSSSEPDTTASWVIHPAETIPTVSKTTPNFFHSELDTVSSTATSHGADVSSAIPTNISPSELDALTPLVTISGTDTSTTFPTLTKSPHETETRTTWLTHPAETSSTIPRTIPNFSHHESDATPSIATSPGAETSSAIPIMTVSPGAEDLVTSQVTSSGTDRNMTIPTLTLSPGEPKTIASLVTHPEAQTSSAIPTSTISPAVSRLVTSMVTSLAAKTSTTNRALTNSPGEPATTVSLVTHPAQTSPTVPWTTSIFFHSKSDTTPSMTTSHGAESSSAVPTPTVSTEVPGVVTPLVTSSRAVISTTIPILTLSPGEPETTPSMATSHGEEASSAIPTPTVSPGVPGVVTSLVTSSRAVTSTTIPILTFSLGEPETTPSMATSHGTEAGSAVPTVLPEVPGMVTSLVASSRAVTSTTLPTLTLSPGEPETTPSMATSHGAEASSTVPTVSPEVPGVVTSLVTSSSGVNSTSIPTLILSPGELETTPSMATSHGAEASSAVPTPTVSPGVSGVVTPLVTSSRAVTSTTIPILTLSSSEPETTPSMATSHGVEASSAVLTVSPEVPGMVTSLVTSSRAVTSTTIPTLTISSDEPETTTSLVTHSEAKMISAIPTLAVSPTVQGLVTSLVTSSGSETSAFSNLTVASSQPETIDSWVAHPGTEASSVVPTLTVSTGEPFTNISLVTHPAESSSTLPRTTSRFSHSELDTMPSTVTSPEAESSSAISTTISPGIPGVLTSLVTSSGRDISATFPTVPESPHESEATASWVTHPAVTSTTVPRTTPNYSHSEPDTTPSIATSPGAEATSDFPTITVSPDVPDMVTSQVTSSGTDTSITIPTLTLSSGEPETTTSFITYSETHTSSAIPTLPVSPGASKMLTSLVISSGTDSTTTFPTLTETPYEPETTAIQLIHPAETNTMVPRTTPKFSHSKSDTTLPVAITSPGPEASSAVSTTTISPDMSDLVTSLVPSSGTDTSTTFPTLSETPYEPETTATWLTHPAETSTTVSGTIPNFSHRGSDTAPSMVTSPGVDTRSGVPTTTIPPSIPGVVTSQVTSSATDTSTAIPTLTPSPGEPETTASSATHPGTQTGFTVPIRTVPSSEPDTMASWVTHPPQTSTPVSRTTSSFSHSSPDATPVMATSPRTEASSAVLTTISPGAPEMVTSQITSSGAATSTTVPTLTHSPGMPETTALLSTHPRTETSKTFPASTVFPQVSETTASLTIRPGAETSTALPTQTTSSLFTLLVTGTSRVDLSPTASPGVSAKTAPLSTHPGTETSTMIPTSTLSLGLLETTGLLATSSSAETSTSTLTLTVSPAVSGLSSASITTDKPQTVTSWNTETSPSVTSVGPPEFSRTVTGTTMTLIPSEMPTPPKTSHGEGVSPTTILRTTMVEATNLATTGSSPTVAKTTTTFNTLAGSLFTPLTTPGMSTLASESVTSRTSYNHRSWISTTSSYNRRYWTPATSTPVTSTFSPGISTSSIPSSTAATVPFMVPFTLNFTITNLQYEEDMRHPGSRKFNATERELQGLLKPLFRNSSLEYLYSGCRLASLRPEKDSSATAVDAICTHRPDPEDLGLDRERLYWELSNLTNGIQELGPYTLDRNSLYVNGFTHRSSMPTTSTPGTSTVDVGTSGTPSSSPSPTTAGPLLMPFTLNFTITNLQYEEDMRRTGSRKFNTMESVLQGLLKPLFKNTSVGPLYSGCRLTLLRPEKDGAATGVDAICTHRLDPKSPGLNREQLYWELSKLTNDIEELGPYTLDRNSLYVNGFTHQSSVSTTSTPGTSTVDLRTSGTPSSLSSPTIMAAGPLLVPFTLNFTITNLQYGEDMGHPGSRKFNTTERVLQGLLGPIFKNTSVGPLYSGCRLTSLRSEKDGAATGVDAICIHHLDPKSPGLNRERLYWELSQLTNGIKELGPYTLDRNSLYVNGFTHRTSVPTSSTPGTSTVDLGTSGTPFSLPSPATAGPLLVLFTLNFTITNLKYEEDMHRPGSRKFNTTERVLQTLLGPMFKNTSVGLLYSGCRLTLLRSEKDGAATGVDAICTHRLDPKSPGVDREQLYWELSQLTNGIKELGPYTLDRNSLYVNGFTHWIPVPTSSTPGTSTVDLGSGTPSSLPSPTTAGPLLVPFTLNFTITNLKYEEDMHCPGSRKFNTTERVLQSLLGPMFKNTSVGPLYSGCRLTLLRSEKDGAATGVDAICTHRLDPKSPGVDREQLYWELSQLTNGIKELGPYTLDRNSLYVNGFTHQTSAPNTSTPGTSTVDLGTSGTPSSLPSPTSAGPLLVPFTLNFTITNLQYEEDMHHPGSRKFNTTERVLQGLLGPMFKNTSVGLLYSGCRLTLLRPEKNGAATGMDAICSHRLDPKSPGLNREQLYWELSQLTHGIKELGPYTLDRNSLYVNGFTHRSSVAPTSTPGTSTVDLGTSGTPSSLPSPTTAVPLLVPFTLNFTITNLQYGEDMRHPGSRKFNTTERVLQGLLGPLFKNSSVGPLYSGCRLISLRSEKDGAATGVDAICTHHLNPQSPGLDREQLYWQLSQMTNGIKELGPYTLDRNSLYVNGFTHRSSGLTTSTPWTSTVDLGTSGTPSPVPSPTTTGPLLVPFTLNFTITNLQYEENMGHPGSRKFNITESVLQGLLKPLFKSTSVGPLYSGCRLTLLRPEKDGVATRVDAICTHRPDPKIPGLDRQQLYWELSQLTHSITELGPYTLDRDSLYVNGFTQRSSVPTTSTPGTFTVQPETSETPSSLPGPTATGPVLLPFTLNFTITNLQYEEDMRRPGSRKFNTTERVLQGLLMPLFKNTSVSSLYSGCRLTLLRPEKDGAATRVDAVCTHRPDPKSPGLDRERLYWKLSQLTHGITELGPYTLDRHSLYVNGFTHQSSMTTTRTPDTSTMHLATSRTPASLSGPMTASPLLVLFTINFTITNLRYEENMHHPGSRKFNTTERVLQGLLRPVFKNTSVGPLYSGCRLTLLRPKKDGAATKVDAICTYRPDPKSPGLDREQLYWELSQLTHSITELGPYTLDRDSLYVNGFTQRSSVPTTSIPGTPTVDLGTSGTPVSKPGPSAASPLLVLFTLNFTITNLRYEENMQHPGSRKFNTTERVLQGLLRSLFKSTSVGPLYSGCRLTLLRPEKDGTATGVDAICTHHPDPKSPRLDREQLYWELSQLTHNITELGPYALDNDSLFVNGFTHRSSVSTTSTPGTPTVYLGASKTPASIFGPSAASHLLILFTLNFTITNLRYEENMWPGSRKFNTTERVLQGLLRPLFKNTSVGPLYSGCRLTLLRPEKDGEATGVDAICTHRPDPTGPGLDREQLYLELSQLTHSITELGPYTLDRDSLYVNGFTHRSSVPTTSTGVVSEEPFTLNFTINNLRYMADMGQPGSLKFNITDNVMQHLLSPLFQRSSLGARYTGCRVIALRSVKNGAETRVDLLCTYLQPLSGPGLPIKQVFHELSQQTHGITRLGPYSLDKDSLYLNGYNEPGPDEPPTTPKPATTFLPPLSEATTAMGYHLKTLTLNFTISNLQYSPDMGKGSATFNSTEGVLQHLLRPLFQKSSMGPFYLGCQLISLRPEKDGAATGVDTTCTYHPDPVGPGLDIQQLYWELSQLTHGVTQLGFYVLDRDSLFINGYAPQNLSIRGEYQINFHIVNWNLSNPDPTSSEYITLLRDIQDKVTTLYKGSQLHDTFRFCLVTNLTMDSVLVTVKALFSSNLDPSLVEQVFLDKTLNASFHWLGSTYQLVDIHVTEMESSVYQPTSSSSTQHFYLNFTITNLPYSQDKAQPGTTNYQRNKRNIEDALNQLFRNSSIKSYFSDCQVSTFRSVPNRHHTGVDSLCNFSPLARRVDRVAIYEEFLRMTRNGTQLQNFTLDRSSVLVDGYSPNRNEPLTGNSDLPFWAVILIGLAGLLGVITCLICGVLVTTRRRKKEGEYNVQQQCPGYYQSHLDLEDLQ

SEQ ID NO: 137 - DNA, 43815 bp, Homo sapiens
  misc_feature 1..43815: note = Immature Human MUC16 nucleic acid sequence (NM_024690.2)
  source 1..43815: mol_type = other DNA
agcgttgcacaattcccccaacctccatacatacggcagctcttctagacacaggttttcccaggtcaaatgcggggaccccagccatatctcccaccctgagaaattttggagtttcagggagctcagaagctctgcagaggccaccctctctgaggggattcttcttagacctccatccagaggcaaatgttgacctgtccatgctgaaaccctcaggccttcctgggtcatcttctcccacccgctccttgatgacagggagcaggagcactaaagccacaccagaaatggattcaggactgacaggagccaccttgtcacctaagacatctacaggtgcaatcgtggtgacagaacatactctgccctttacttccccagataagaccttggccagtcctacatcttcggttgtgggaagaaccacccagtctttgggggtgatgtcctctgctctccctgagtcaacctctagaggaatgacacactccgagcaaagaaccagcccatcgctgagtccccaggtcaatggaactccctctaggaactaccctgctacaagcatggtttcaggattgagttccccaaggaccaggaccagttccacagaaggaaattttaccaaagaagcatctacatacacactcactgtagagaccacaagtggcccagtcactgagaagtacacagtccccactgagacctcaacaactgaaggtgacagcacagagaccccctgggacacaagatatattcctgtaaaaatcacatctccaatgaaaacatttgcagattcaactgcatccaaggaaaatgccccagtgtctatgactccagctgagaccacagttactgactcacatactccaggaaggacaaacccatcatttgggacactttattcttccttccttgacctatcacctaaagggaccccaaattccagaggtgaaacaagcctggaactgattctatcaaccactggatatcccttctcctctcctgaacctggctctgcaggacacagcagaataagtaccagtgcgcctttgtcatcatctgcttcagttctcgataataaaatatcagagaccagcatattctcaggccagagtctcacctcccctctgtctcctggggtgcccgaggccagagccagcacaatgcccaactcagctatccctttttccatgacactaagcaatgcagaaacaagtgccgaaagggtcagaagcacaatttcctctctggggactccatcaatatccacaaagcagacagcagagactatccttaccttccatgccttcgctgagaccatggatatacccagcacccacatagccaagactttggcttcagaatggttgggaagtccaggtacccttggtggcaccagcacttcagcgctgacaaccacatctccatctaccactttagtctcagaggagaccaacacccatcactccacgagtggaaaggaaacagaaggaactttgaatacatctatgactccacttgagacctctgctcctggagaagagtccgaaatgactgccaccttggtccccactctaggttttacaactcttgacagcaagatcagaagtccatctcaggtctcttcatcccacccaacaagagagctcagaaccacaggcagcacctctgggaggcagagttccagcacagctgcccacgggagctctgacatcctgagggcaaccacttccagcacctcaaaagcatcatcatggaccagtgaaagcacagctcagcaatttagtgaaccccagcacacacagtgggtggagacaagtcctagcatgaaaacagagagacccccagcatcaaccagtgtggcagcccctatcaccacttctgttccctcagtggtctctggcttcaccaccctgaagaccagctccacaaaagggatttggcttgaagaaacatctgcagacacactcatcggagaatccacagctggcccaaccacccatcagtttgctgttcccactgggatttcaatgacaggaggcagcagcaccaggggaagccagggcacaacccacctactcaccagagccacagcatcatctgagacatccgcagatttgactctggccacgaacggtgtcccagtctccgtgtctccagcagtgagcaagacggctgctggctcaagtcctccaggagggacaaagccatcatatacaatggtttcttctgtcatccctgagacatcatctctacagtcctcagctttcagggaaggaaccagcctgggactgactccattaaacactagacatcccttctcttcccctgaaccagactctgcaggacacaccaagataagcaccagcattcctctgttgtcatctgcttcagttcttgaggataaagtgtcagcgaccagcacattctcacaccacaaagccacctcatctattaccacagggactcctgaaatctcaacaaagacaaagcccagctcagccgttctttcctccatgaccctaagcaatgcagcaacaagtcctgaaagagtcagaaatgcaacttcccctctgactcatccatctccatcaggggaagagacagcagggagtgtcctcactctcagcacctctgctgagactacagactcacctaacatccacccaactgggacactgacttcagaatcgtcagagagtcctagcactctcagcctcccaagtgtctctggagtcaaaaccacattttcttcatctactccttccactcatctatttactagtggagaagaaacagaggaaacttcgaatccatctgtgtctcaacctgagacttctgtttccagagtaaggaccaccttggccagcacctctgtccctaccccagtattccccaccatggacacctggcctacacgttcagctcagttctcttcatcccacctagtgagtgagctcagagctacgagcagtacctcagttacaaactcaactggttcagctcttcctaaaatatctcacctcactgggacggcaacaatgtcacagaccaatagagacacgtttaatgactctgctgcaccccaaagcacaacttggccagagactagtcccagattcaagacagggttaccttcagcaacaaccactgtttcaacctctgccacttctctctctgctactgtaatggtctctaaattcacttctccagcaactagttccatggaagcaacttctatcagggaaccatcaacaaccatcctcacaacagagaccacgaatggcccaggctctatggctgtggcttctaccaacatcccaattggaaagggctacattactgaaggaagattggacacaagccatctgcccattggaaccacagcttcctctgagacatctatggattttaccatggccaaagaaagtgtctcaatgtcagtatctccatctcagtccatggatgctgctggctcaagcactccaggaaggacaagccaattcgttgacacattttctgatgatgtctatcatttaacatccagagaaattacaatacctagagatggaacaagctcagctctgactccacaaatgactgcaactcaccctccatctcctgatcctggctctgctagaagcacctggcttggcatcttgtcctcatctccttcttctcctactcccaaagtcacaatgagctccacattttcaactcagagagtcaccacaagcatgataatggacacagttgaaactagtcggtggaacatgcccaacttaccttccacgacttccttgacaccaagtaatattccaacaagtggtgccataggaaaaagcaccctggttcccttggacactccatctccagccacatcattggaggcatcagaagggggacttccaaccctcagcacctaccctgaatcaacaaacacacccagcatccacctcggagcacacgctagttcagaaagtccaagcaccatcaaacttaccatggcttcagtagtaaaacctggctcttacacacctctcaccttcccctcaatagagacccacattcatgtatcaacagccagaatggcttactcttctgggtcttcacctgagatgacagctcctggagagactaacactggtagtacctgggaccccaccacctacatcaccactacggatcctaaggatacaagttcagctcaggtctctacaccccactcagtgaggacactcagaaccacagaaaaccatccaaagacagagtccgccaccccagctgcttactctggaagtcctaaaatctcaagttcacccaatctcaccagtccggccacaaaagcatggaccatcacagacacaactgaacactccactcaattacattacacaaaattggcagaaaaatcatctggatttgagacacagtcagctccaggacctgtctctgtagtaatccctacctcccctaccattggaagcagcacattggaactaacttctgatgtcccaggggaacccctggtccttgctcccagtgagcagaccacaatcactctccccatggcaacatggctgagtaccagtttgacagaggaaatggcttcaacagaccttgatatttcaagtccaagttcacccatgagtacatttgctatttttccacctatgtccacaccttctcatgaactttcaaagtcagaggcagataccagtgccattagaaatacagattcaacaacgttggatcagcacctaggaatcaggagtttgggcagaactggggacttaacaactgttcctatcaccccactgacaaccacgtggaccagtgtgattgaacactcaacacaagcacaggacaccctttctgcaacgatgagtcctactcacgtgacacagtcactcaaagatcaaacatctataccagcctcagcatccccttcccatcttactgaagtctaccctgagctcgggacacaagggagaagctcctctgaggcaaccactttttggaaaccatctacagacacactgtccagagagattgagactggcccaacaaacattcaatccactccacccatggacaacacaacaacagggagcagtagtagtggagtcaccctgggcatagcccaccttcccataggaacatcctccccagctgagacatccacaaacatggcactggaaagaagaagttctacagccactgtctctatggctgggacaatgggactccttgttactagtgctccaggaagaagcatcagccagtcattaggaagagtttcctctgtcctttctgagtcaactactgaaggagtcacagattctagtaagggaagcagcccaaggctgaacacacagggaaatacagctctctcctcctctcttgaacccagctatgctgaaggaagccagatgagcacaagcatccctctaacctcatctcctacaactcctgatgtggaattcatagggggcagcacattttggaccaaggaggtcaccacagttatgacctcagacatctccaagtcttcagcaaggacagagtccagctcagctacccttatgtccacagctttgggaagcactgaaaatacaggaaaagaaaaactcagaactgcctctatggatcttccatctccaactccatcaatggaggtgacaccatggatttctctcactctcagtaatgcccccaataccacagattcacttgacctcagccatggggtgcacaccagctctgcagggactttggccactgacaggtcattgaatactggtgtcactagagcctccagattggaaaacggctctgatacctcttctaagtccctgtctatgggaaacagcactcacacttccatgacttacacagagaagagtgaagtgtcttcttcaatccatccccgacctgagacctcagctcctggagcagagaccactttgacttccactcctggaaacagggccataagcttaacattgcctttttcatccattccagtggaagaagtcatttctacaggcataacctcaggaccagacatcaactcagcacccatgacacattctcccatcaccccaccaacaattgtatggaccagtacaggcacaattgaacagtccactcaaccactacatgcagtttcttcagaaaaagtttctgtgcagacacagtcaactccatatgtcaactctgtggcagtgtctgcttcccctacccatgagaattcagtctcttctggaagcagcacatcctctccatattcctcagcctcacttgaatccttggattccacaatcagtaggaggaatgcaatcacttcctggctatgggacctcactacatctctccccactacaacttggccaagtactagtttatctgaggcactgtcctcaggccattctggggtttcaaacccaagttcaactacgactgaatttccactcttttcagctgcatccacatctgctgctaagcaaagaaatccagaaacagagacccatggtccccagaatacagccgcgagtactttgaacactgatgcatcctcggtcacaggtctttctgagactcctgtgggggcaagtatcagctctgaagtccctcttccaatggccataacttctagatcagatgtttctggccttacatctgagagtactgctaacccgagtttaggcacagcctcttcagcagggaccaaattaactaggacaatatccctgcccacttcagagtctttggtttcctttagaatgaacaaggatccatggacagtgtcaatccctttggggtcccatccaactactaatacagaaacaagcatcccagtaaacagcgcaggtccacctggcttgtccacagtagcatcagatgtaattgacacaccttcagatggggctgagagtattcccactgtctccttttccccctcccctgatactgaagtgacaactatctcacatttcccagaaaagacaactcattcatttagaaccatttcatctctcactcatgagttgacttcaagagtgacacctattcctggggattggatgagttcagctatgtctacaaagcccacaggagccagtccctccattacactgggagagagaaggacaatcacctctgctgctccaaccacttcccccatagttctcactgctagtttcacagagaccagcacagtttcactggataatgaaactacagtaaaaacctcagatatccttgacgcacggaaaacaaatgagctcccctcagatagcagttcttcttctgatctgatcaacacctccatagcttcttcaactatggatgtcactaaaacagcctccatcagtcccactagcatctcaggaatgacagcaagttcctccccatctctcttctcttcagatagaccccaggttcccacatctacaacagagacaaatacagccacctctccatctgtttccagtaacacctattctcttgatgggggctccaatgtgggtggcactccatccactttaccaccctttacaatcacccaccctgtcgagacaagctcggccctattagcctggtctagaccagtaagaactttcagcaccatggtcagcactgacactgcctccggagaaaatcctacctctagcaattctgtggtgacttctgttccagcaccaggtacatggaccagtgtaggcagtactactgacttacctgccatgggctttctcaagacaagtcctgcaggagaggcacactcacttctagcatcaactattgaaccagccactgccttcactccccatctctcagcagcagtggtcactggatccagtgctacatcagaagccagtcttctcactacgagtgaaagcaaagccattcattcttcaccacagaccccaactacacccacctctggagcaaactgggaaacttcagctactcctgagagccttttggtagtcactgagacttcagacacaacacttacctcaaagattttggtcacagataccatcttgttttcaactgtgtccacgccaccttctaaatttccaagtacggggactctgtctggagcttccttccctactttactcccggacactccagccatccctctcactgccactgagccaacaagttcattagctacatcctttgattccaccccactggtgactatagcttcggatagtcttggcacagtcccagagactaccctgaccatgtcagagacctcaaatggtgatgcactggttcttaagacagtaagtaacccagataggagcatccctggaatcactatccaaggagtaacagaaagtccactccatccttcttccacttccccctctaagattgttgctccacggaatacaacctatgaaggttcgatcacagtggcactttctactttgcctgcgggaactactggttcccttgtattcagtcagagttctgaaaactcagagacaacggctttggtagactcatcagctgggcttgagagggcatctgtgatgccactaaccacaggaagccagggtatggctagctctggaggaatcagaagtgggtccactcactcaactggaaccaaaacattttcttctctccctctgaccatgaacccaggtgaggttacagccatgtctgaaatcaccacgaacagactgacagctactcaatcaacagcacccaaagggatacctgtgaagcccaccagtgctgagtcaggcctcctaacacctgtctctgcctcctcaagcccatcaaaggcctttgcctcactgactacagctcccccaacttgggggatcccacagtctaccttgacatttgagttttctgaggtcccaagtttggatactaagtccgcttctttaccaactcctggacagtccctgaacaccattccagactcagatgcaagcacagcatcttcctcactgtccaagtctccagaaaaaaacccaagggcaaggatgatgacttccacaaaggccataagtgcaagctcatttcaatcaacaggttttactgaaacccctgagggatctgcctccccttctatggcagggcatgaacccagagtccccacttcaggaacaggggaccctagatatgcctcagagagcatgtcttatccagacccaagcaaggcatcatcagctatgacatcgacctctcttgcatcaaaactcacaactctcttcagcacaggtcaagcagcaaggtctggttctagttcctctcccataagcctatccactgagaaagaaacaagcttcctttcccccactgcatccacctccagaaagacttcactatttcttgggccttccatggcaaggcagcccaacatattggtgcatcttcagacttcagctctgacactttctccaacatccactctaaatatgtcccaggaggagcctcctgagttaacctcaagccagaccattgcagaagaagagggaacaacagctgaaacacagacgttaaccttcacaccatctgagaccccaacatccttgttacctgtctcttctcccacagaacccacagccagaagaaagagttctccagaaacatgggcaagctctatttcagttcctgccaagacctccttggttgaaacaactgatggaacgctagtgaccaccataaagatgtcaagccaggcagcacaaggaaattccacgtggcctgccccagcagaggagacggggagcagtccagcaggcacatccccaggaagcccagaaatgtctaccactctcaaaatcatgagctccaaggaacccagcatcagcccagagatcaggtccactgtgagaaattctccttggaagactccagaaacaactgttcccatggagaccacagtggaaccagtcacccttcagtccacagccctaggaagtggcagcaccagcatctctcacctgcccacaggaaccacatcaccaaccaagtcaccaacagaaaatatgttggctacagaaagggtctccctctccccatccccacctgaggcttggaccaacctttattctggaactccaggagggaccaggcagtcactggccacaatgtcctctgtctccctagagtcaccaactgctagaagcatcacagggactggtcagcaaagcagtccagaactggtttcaaagacaactggaatggaattctctatgtggcatggctctactggagggaccacaggggacacacatgtctctctgagcacatcttccaatatccttgaagaccctgtaaccagcccaaactctgtgagctcattgacagataaatccaaacataaaaccgagacatgggtaagcaccacagccattccctccactgtcctgaataataagataatggcagctgaacaacagacaagtcgatctgtggatgaggcttattcatcaactagttcttggtcagatcagacatctgggagtgacatcacccttggtgcatctcctgatgtcacaaacacattatacatcacctccacagcacaaaccacctcactagtgtctctgccctctggagaccaaggcattacaagcctcaccaatccctcaggaggaaaaacaagctctgcgtcatctgtcacatctccttcaatagggcttgagactctgagggccaatgtaagtgcagtgaaaagtgacattgcccctactgctgggcatctatctcagacttcatctcctgcggaagtgagcatcctggacgtaaccacagctcctactccaggtatctccaccaccatcaccaccatgggaaccaactcaatctcaactaccacacccaacccagaagtgggtatgagtaccatggacagcaccccggccacagagaggcgcacaacttctacagaacacccttccacctggtcttccacagctgcatcagattcctggactgtcacagacatgacttcaaacttgaaagttgcaagatctcctggaacaatttccacaatgcatacaacttcattcttagcctcaagcactgaattagactccatgtctactccccatggccgtataactgtcattggaaccagcctggtcactccatcctctgatgcttcagctgtaaagacagagaccagtacaagtgaaagaacattgagtccttcagacacaactgcatctactcccatctcaactttttctcgtgtccagaggatgagcatctcagttcctgacattttaagtacaagttggactcccagtagtacagaagcagaagatgtgcctgtttcaatggtttctacagatcatgctagtacaaagactgacccaaatacgcccctgtccacttttctgtttgattctctgtccactcttgactgggacactgggagatctctgtcatcagccacagccactacctcagctcctcagggggccacaactccccaggaactcactttggaaaccatgatcagcccagctacctcacagttgcccttctctatagggcacattacaagtgcagtcacaccagctgcaatggcaaggagctctggagttactttttcaagaccagatcccacaagcaaaaaggcagagcagacttccactcagcttcccaccaccacttctgcacatccagggcaggtgcccagatcagcagcaacaactctggatgtgatcccacacacagcaaaaactccagatgcaacttttcagagacaagggcagacagctcttacaacagaggcaagagctacatctgactcctggaatgagaaagaaaaatcaaccccaagtgcaccttggatcactgagatgatgaattctgtctcagaagataccatcaaggaggttaccagctcctccagtgtattaaggaccctgaatacgctggacataaacttggaatctgggacgacttcatccccaagttggaaaagcagcccatatgagagaattgccccttctgagtccaccacagacaaagaggcaattcacccttctacaaacacagtagagaccacaggctgggtcacaagttccgaacatgcttctcattccactatcccagcccactcagcgtcatccaaactcacatctccagtggttacaacctccaccagggaacaagcaatagtttctatgtcaacaaccacatggccagagtctacaagggctagaacagagcctaattccttcttgactattgaactgagggacgtcagcccttacatggacaccagctcaaccacacaaacaagtattatctcttccccaggttccactgcgatcaccaaggggcctagaacagaaattacctcctctaagagaatatccagctcattccttgcccagtctatgaggtcgtcagacagcccctcagaagccatcaccaggctgtctaactttcctgccatgacagaatctggaggaatgatccttgctatgcaaacaagtccacctggcgctacatcactaagtgcacctactttggatacatcagccacagcctcctggacagggactccactggctacgactcagagatttacatactcagagaagaccactctctttagcaaaggtcctgaggatacatcacagccaagccctccctctgtggaagaaaccagctcttcctcttccctggtacctatccatgctacaacctcgccttccaatattttgttgacatcacaagggcacagtccctcctctactccacctgtgacctcagttttcttgtctgagacctctggcctggggaagaccacagacatgtcgaggataagcttggaacctggcacaagtttacctcccaatttgagcagtacagcaggtgaggcgttatccacttatgaagcctccagagatacaaaggcaattcatcattctgcagacacagcagtgacgaatatggaggcaaccagttctgaatattctcctatcccaggccatacaaagccatccaaagccacatctccattggttacctcccacatcatgggggacatcacttcttccacatcagtatttggctcctccgagaccacagagattgagacagtgtcctctgtgaaccagggacttcaggagagaagcacatcccaggtggccagctctgctacagagacaagcactgtcattacccatgtgtctagtggtgatgctactactcatgtcaccaagacacaagccactttctctagcggaacatccatctcaagccctcatcagtttataacttctaccaacacatttacagatgtgagcaccaacccctccacctctctgataatgacagaatcttcaggagtgaccatcaccacccaaacaggtcctactggagctgcaacacagggtccatatctcttggacacatcaaccatgccttacttgacagagactccattagctgtgactccagattttatgcaatcagagaagaccactctcataagcaaaggtcccaaggatgtgtcctggacaagccctccctctgtggcagaaaccagctatccctcttccctgacacctttcttggtcacaaccatacctcctgccacttccacgttacaagggcaacatacatcctctcctgtttctgcgacttcagttcttacctctggactggtgaagaccacagatatgttgaacacaagcatggaacctgtgaccaattcacctcaaaatttgaacaatccatcaaatgagatactggccactttggcagccaccacagatatagagactattcatccttccataaacaaagcagtgaccaatatggggactgccagttcagcacatgtactgcattccactctcccagtcagctcagaaccatctacagccacatctccaatggttcctgcctccagcatgggggacgctcttgcttctatatcaatacctggttctgagaccacagacattgagggagagccaacatcctccctgactgctggacgaaaagagaacagcaccctccaggagatgaactcaactacagagtcaaacatcatcctctccaatgtgtctgtgggggctattactgaagccacaaaaatggaagtcccctcttttgatgcaacattcataccaactcctgctcagtcaacaaagttcccagatattttctcagtagccagcagtagactttcaaactctcctcccatgacaatatctacccacatgaccaccacccagacagggtcttctggagctacatcaaagattccacttgccttagacacatcaaccttggaaacctcagcagggactccatcagtggtgactgaggggtttgcccactcaaaaataaccactgcaatgaacaatgatgtcaaggacgtgtcacagacaaaccctccctttcaggatgaagccagctctccctcttctcaagcacctgtccttgtcacaaccttaccttcttctgttgctttcacaccgcaatggcacagtacctcctctcctgtttctatgtcctcagttcttacttcttcactggtaaagaccgcaggcaaggtggatacaagcttagaaacagtgaccagttcacctcaaagtatgagcaacactttggatgacatatcggtcacttcagcagccaccacagatatagagacaacgcatccttccataaacacagtagttaccaatgtggggaccaccggttcagcatttgaatcacattctactgtctcagcttacccagagccatctaaagtcacatctccaaatgttaccacctccaccatggaagacaccacaatttccagatcaatacctaaatcctctaagactacaagaactgagactgagacaacttcctccctgactcctaaactgagggagaccagcatctcccaggagatcacctcgtccacagagacaagcactgttccttacaaagagctcactggtgccactaccgaggtatccaggacagatgtcacttcctctagcagtacatccttccctggccctgatcagtccacagtgtcactagacatctccacagaaaccaacaccaggctgtctacctccccaataatgacagaatctgcagaaataaccatcaccacccaaacaggtcctcatggggctacatcacaggatacttttaccatggacccatcaaatacaaccccccaggcagggatccactcagctatgactcatggattttcacaattggatgtgaccactcttatgagcagaattccacaggatgtatcatggacaagtcctccctctgtggataaaaccagctccccctcttcctttctgtcctcacctgcaatgaccacaccttccctgatttcttctaccttaccagaggataagctctcctctcctatgacttcacttctcacctctggcctagtgaagattacagacatattacgtacacgcttggaacctgtgaccagctcacttccaaatttcagcagcacctcagataagatactggccacttctaaagacagtaaagacacaaaggaaatttttccttctataaacacagaagagaccaatgtgaaagccaacaactctggacatgaatcccattcccctgcactggctgactcagagacacccaaagccacaactcaaatggttatcaccaccactgtgggagatccagctccttccacatcaatgccagtgcatggttcctctgagactacaaacattaagagagagccaacatatttcttgactcctagactgagagagaccagtacctctcaggagtccagctttcccacggacacaagttttctactttccaaagtccccactggtactattactgaggtctccagtacaggggtcaactcttctagcaaaatttccaccccagaccatgataagtccacagtgccacctgacaccttcacaggagagatccccagggtcttcacctcctctattaagacaaaatctgcagaaatgacgatcaccacccaagcaagtcctcctgagtctgcatcgcacagtacccttcccttggacacatcaaccacactttcccagggagggactcattcaactgtgactcagggattcccatactcagaggtgaccactctcatgggcatgggtcctgggaatgtgtcatggatgacaactccccctgtggaagaaaccagctctgtgtcttccctgatgtcttcacctgccatgacatccccttctcctgtttcctccacatcaccacagagcatcccctcctctcctcttcctgtgactgcacttcctacttctgttctggtgacaaccacagatgtgttgggcacaacaagcccagagtctgtaaccagttcacctccaaatttgagcagcatcactcatgagagaccggccacttacaaagacactgcacacacagaagccgccatgcatcattccacaaacaccgcagtgaccaatgtagggacttccgggtctggacataaatcacaatcctctgtcctagctgactcagagacatcgaaagccacacctctgatgagtaccacctccaccctgggggacacaagtgtttccacatcaactcctaatatctctcagactaaccaaattcaaacagagccaacagcatccctgagccctagactgagggagagcagcacgtctgagaagaccagctcaacaacagagacaaatactgccttttcttatgtgcccacaggtgctattactcaggcctccagaacagaaatctcctctagcagaacatccatctcagaccttgatcggcccacaatagcacccgacatctccacaggaatgatcaccaggctcttcacctcccccatcatgacaaaatctgcagaaatgaccgtcaccactcaaacaactactcctggggctacatcacagggtatccttccctgggacacatcaaccacacttttccagggagggactcattcaaccgtgtctcagggattcccacactcagagataaccactcttcggagcagaacccctggagatgtgtcatggatgacaactccccctgtggaagaaaccagctctgggttttccctgatgtcaccttccatgacatccccttctcctgtttcctccacatcaccagagagcatcccctcctctcctctccctgtgactgcacttcttacttctgttctggtgacaaccacaaatgtattgggcacaacaagcccagagcccgtaacgagttcacctccaaatttaagcagccccacacaggagagactgaccacttacaaagacactgcgcacacagaagccatgcatgcttccatgcatacaaacactgcagtggccaacgtggggacctccatttctggacatgaatcacaatcttctgtcccagctgattcacacacatccaaagccacatctccaatgggtatcaccttcgccatgggggatacaagtgtttctacatcaactcctgccttctttgagactagaattcagactgaatcaacatcctctttgattcctggattaagggacaccaggacgtctgaggagatcaacactgtgacagagaccagcactgtcctttcagaagtgcccactactactactactgaggtctccaggacagaagttatcacttccagcagaacaaccatctcagggcctgatcattccaaaatgtcaccctacatctccacagaaaccatcaccaggctctccacttttccttttgtaacaggatccacagaaatggccatcaccaaccaaacaggtcctatagggactatctcacaggctacccttaccctggacacatcaagcacagcttcctgggaagggactcactcacctgtgactcagagatttccacactcagaggagaccactactatgagcagaagtactaagggcgtgtcatggcaaagccctccctctgtggaagaaaccagttctccttcttccccagtgcctttacctgcaataacctcacattcatctctttattccgcagtatcaggaagtagccccacttctgctctccctgtgacttcccttctcacctctggcaggaggaagaccatagacatgttggacacacactcagaacttgtgaccagctccttaccaagtgcaagtagcttctcaggtgagatactcacttctgaagcctccacaaatacagagacaattcacttttcagagaacacagcagaaaccaatatggggaccaccaattctatgcataaactacattcctctgtctcaatccactcccagccatccggacacacacctccaaaggttactggatctatgatggaggacgctattgtttccacatcaacacctggttctcctgagactaaaaatgttgacagagactcaacatcccctctgactcctgaactgaaagaggacagcaccgccctggtgatgaactcaactacagagtcaaacactgttttctccagtgtgtccctggatgctgctactgaggtctccagggcagaagtcacctactatgatcctacattcatgccagcttctgctcagtcaacaaagtccccagacatttcacctgaagccagcagcagtcattctaactctcctcccttgacaatatctacacacaagaccatcgccacacaaacaggtccttctggggtgacatctcttggccaactgaccctggacacatcaaccatagccacctcagcaggaactccatcagccagaactcaggattttgtagattcagaaacaaccagtgtcatgaacaatgatctcaatgatgtgttgaagacaagccctttctctgcagaagaagccaactctctctcttctcaggcacctctccttgtgacaacctcaccttctcctgtaacttccacattgcaagagcacagtacctcctctcttgtttctgtgacctcagtacccacccctacactggcgaagatcacagacatggacacaaacttagaacctgtgactcgttcacctcaaaatttaaggaacaccttggccacttcagaagccaccacagatacacacacaatgcatccttctataaacacagcagtggccaatgtggggaccaccagttcaccaaatgaattctattttactgtctcacctgactcagacccatataaagccacatccgcagtagttatcacttccacctcgggggactcaatagtttccacatcaatgcctagatcctctgcgatgaaaaagattgagtctgagacaactttctccctgatatttagactgagggagactagcacctcccagaaaattggctcatcctcagacacaagcacggtctttgacaaagcattcactgctgctactactgaggtctccagaacagaactcacctcctctagcagaacatccatccaaggcactgaaaagcccacaatgtcaccggacacctccacaagatctgtcaccatgctttctacttttgctggcctgacaaaatccgaagaaaggaccattgccacccaaacaggtcctcatagggcgacatcacagggtacccttacctgggacacatcaatcacaacctcacaggcagggacccactcagctatgactcatggattttcacaattagatttgtccactcttacgagtagagttcctgagtacatatcagggacaagcccaccctctgtggaaaaaaccagctcttcctcttcccttctgtctttaccagcaataacctcaccgtcccctgtacctactacattaccagaaagtaggccgtcttctcctgttcatctgacttcactccccacctctggcctagtgaagaccacagatatgctggcatctgtggccagtttacctccaaacttgggcagcacctcacataagataccgactacttcagaagacattaaagatacagagaaaatgtatccttccacaaacatagcagtaaccaatgtggggaccaccacttctgaaaaggaatcttattcgtctgtcccagcctactcagaaccacccaaagtcacctctccaatggttacctctttcaacataagggacaccattgtttccacatccatgcctggctcctctgagattacaaggattgagatggagtcaacattctccctggctcatgggctgaagggaaccagcacctcccaggaccccatcgtatccacagagaaaagtgctgtccttcacaagttgaccactggtgctactgagacctctaggacagaagttgcctcttctagaagaacatccattccaggccctgatcattccacagagtcaccagacatctccactgaagtgatccccagcctgcctatctcccttggcattacagaatcttcaaatatgaccatcatcactcgaacaggtcctcctcttggctctacatcacagggcacatttaccttggacacaccaactacatcctccagggcaggaacacactcgatggcgactcaggaatttccacactcagaaatgaccactgtcatgaacaaggaccctgagattctatcatggacaatccctccttctatagagaaaaccagcttctcctcttccctgatgccttcaccagccatgacttcacctcctgtttcctcaacattaccaaagaccattcacaccactccttctcctatgacctcactgctcacccctagcctagtgatgaccacagacacattgggcacaagcccagaacctacaaccagttcacctccaaatttgagcagtacctcacatgagatactgacaacagatgaagacaccacagctatagaagccatgcatccttccacaagcacagcagcgactaatgtggaaaccaccagttctggacatgggtcacaatcctctgtcctagctgactcagaaaaaaccaaggccacagctccaatggataccacctccaccatggggcatacaactgtttccacatcaatgtctgtttcctctgagactacaaaaattaagagagagtcaacatattccttgactcctggactgagagagaccagcatttcccaaaatgccagcttttccactgacacaagtattgttctttcagaagtccccactggtactactgctgaggtctccaggacagaagtcacctcctctggtagaacatccatccctggcccttctcagtccacagttttgccagaaatatccacaagaacaatgacaaggctctttgcctcgcccaccatgacagaatcagcagaaatgaccatccccactcaaacaggtccttctgggtctacctcacaggatacccttaccttggacacatccaccacaaagtcccaggcaaagactcattcaactttgactcagagatttccacactcagagatgaccactctcatgagcagaggtcctggagatatgtcatggcaaagctctccctctctggaaaatcccagctctctcccttccctgctgtctttacctgccacaacctcacctcctcccatttcctccacattaccagtgactatctcctcctctcctcttcctgtgacttcacttctcacctctagcccggtaacgaccacagacatgttacacacaagcccagaacttgtaaccagttcacctccaaagctgagccacacttcagatgagagactgaccactggcaaggacaccacaaatacagaagctgtgcatccttccacaaacacagcagcgtccaatgtggagattcccagctctggacatgaatccccttcctctgccttagctgactcagagacatccaaagccacatcaccaatgtttattacctccacccaggaggatacaactgttgccatatcaacccctcacttcttggagactagcagaattcagaaagagtcaatttcctccctgagccctaaattgagggagacaggcagttctgtggagacaagctcagccatagagacaagtgctgtcctttctgaagtgtccattggtgctactactgagatctccaggacagaagtcacctcctctagcagaacatccatctctggttctgctgagtccacaatgttgccagaaatatccaccacaagaaaaatcattaagttccctacttcccccatcctggcagaatcatcagaaatgaccatcaagacccaaacaagtcctcctgggtctacatcagagagtacctttacattagacacatcaaccactccctccttggtaataacccattcgactatgactcagagattgccacactcagagataaccactcttgtgagtagaggtgctggggatgtgccacggcccagctctctccctgtggaagaaacaagccctccatcttcccagctgtctttatctgccatgatctcaccttctcctgtttcttccacattaccagcaagtagccactcctcttctgcttctgtgacttcacttctcacaccaggccaagtgaagactactgaggtgttggacgcaagtgcagaacctgaaaccagttcacctccaagtttgagcagcacctcagttgaaatactggccacctctgaagtcaccacagatacggagaaaattcatcctttctcaaacacggcagtaaccaaagttggaacttccagttctggacatgaatccccttcctctgtcctacctgactcagagacaaccaaagccacatcggcaatgggtaccatctccattatgggggatacaagtgtttctacattaactcctgccttatctaacactaggaaaattcagtcagagccagcttcctcactgaccaccagattgagggagaccagcacctctgaagagaccagcttagccacagaagcaaacactgttctttctaaagtgtccactggtgctactactgaggtctccaggacagaagccatctcctttagcagaacatccatgtcaggccctgagcagtccacaatgtcacaagacatctccataggaaccatccccaggatttctgcctcctctgtcctgacagaatctgcaaaaatgaccatcacaacccaaacaggtccttcggagtctacactagaaagtacccttaatttgaacacagcaaccacaccctcttgggtggaaacccactctatagtaattcagggatttccacacccagagatgaccacttccatgggcagaggtcctggaggtgtgtcatggcctagccctccctttgtgaaagaaaccagccctccatcctccccgctgtctttacctgccgtgacctcacctcatcctgtttccaccacattcctagcacatatccccccctctccccttcctgtgacttcacttctcacctctggcccggcgacaaccacagatatcttgggtacaagcacagaacctggaaccagttcatcttcaagtttgagcaccacctcccatgagagactgaccacttacaaagacactgcacatacagaagccgtgcatccttccacaaacacaggagggaccaatgtggcaaccaccagctctggatataaatcacagtcctctgtcctagctgactcatctccaatgtgtaccacctccaccatgggggatacaagtgttctcacatcaactcctgccttccttgagactaggaggattcagacagagctagcttcctccctgacccctggattgagggagtccagcggctctgaagggaccagctcaggcaccaagatgagcactgtcctctctaaagtgcccactggtgctactactgagatctccaaggaagacgtcacctccatcccaggtcccgctcaatccacaatatcaccagacatctccacaagaaccgtcagctggttctctacatcccctgtcatgacagaatcagcagaaataaccatgaacacccatacaagtcctttaggggccacaacacaaggcaccagtactttggacacgtcaagcacaacctctttgacaatgacacactcaactatatctcaaggattttcacactcacagatgagcactcttatgaggaggggtcctgaggatgtatcatggatgagccctccccttctggaaaaaactagaccttccttttctctgatgtcttcaccagccacaacttcaccttctcctgtttcctccacattaccagagagcatctcttcctctcctcttcctgtgacttcactcctcacgtctggcttggcaaaaactacagatatgttgcacaaaagctcagaacctgtaaccaactcacctgcaaatttgagcagcacctcagttgaaatactggccacctctgaagtcaccacagatacagagaaaactcatccttcttcaaacagaacagtgaccgatgtggggacctccagttctggacatgaatccacttcctttgtcctagctgactcacagacatccaaagtcacatctccaatggttattacctccaccatggaggatacgagtgtctccacatcaactcctggcttttttgagactagcagaattcagacagaaccaacatcctccctgacccttggactgagaaagaccagcagctctgaggggaccagcttagccacagagatgagcactgtcctttctggagtgcccactggtgccactgctgaagtctccaggacagaagtcacctcctctagcagaacatccatctcaggctttgctcagctcacagtgtcaccagagacttccacagaaaccatcaccagactccctacctccagcataatgacagaatcagcagaaatgatgatcaagacacaaacagatcctcctgggtctacaccagagagtactcatactgtggacatatcaacaacacccaactgggtagaaacccactcgactgtgactcagagattttcacactcagagatgaccactcttgtgagcagaagccctggtgatatgttatggcctagtcaatcctctgtggaagaaaccagctctgcctcttccctgctgtctctgcctgccacgacctcaccttctcctgtttcctctacattagtagaggatttcccttccgcttctcttcctgtgacttctcttctcaaccctggcctggtgataaccacagacaggatgggcataagcagagaacctggaaccagttccacttcaaatttgagcagcacctcccatgagagactgaccactttggaagacactgtagatacagaagacatgcagccttccacacacacagcagtgaccaacgtgaggacctccatttctggacatgaatcacaatcttctgtcctatctgactcagagacacccaaagccacatctccaatgggtaccacctacaccatgggggaaacgagtgtttccatatccacttctgacttctttgagaccagcagaattcagatagaaccaacatcctccctgacttctggattgagggagaccagcagctctgagaggatcagctcagccacagagggaagcactgtcctttctgaagtgcccagtggtgctaccactgaggtctccaggacagaagtgatatcctctaggggaacatccatgtcagggcctgatcagttcaccatatcaccagacatctctactgaagcgatcaccaggctttctacttcccccattatgacagaatcagcagaaagtgccatcactattgagacaggttctcctggggctacatcagagggtaccctcaccttggacacctcaacaacaaccttttggtcagggacccactcaactgcatctccaggattttcacactcagagatgaccactcttatgagtagaactcctggagatgtgccatggccgagccttccctctgtggaagaagccagctctgtctcttcctcactgtcttcacctgccatgacctcaacttcttttttctccacattaccagagagcatctcctcctctcctcatcctgtgactgcacttctcacccttggcccagtgaagaccacagacatgttgcgcacaagctcagaacctgaaaccagttcacctccaaatttgagcagcacctcagctgaaatattagccacgtctgaagtcaccaaagatagagagaaaattcatccctcctcaaacacacctgtagtcaatgtagggactgtgatttataaacatctatccccttcctctgttttggctgacttagtgacaacaaaacccacatctccaatggctaccacctccactctggggaatacaagtgtttccacatcaactcctgccttcccagaaactatgatgacacagccaacttcctccctgacttctggattaagggagatcagtacctctcaagagaccagctcagcaacagagagaagtgcttctctttctggaatgcccactggtgctactactaaggtctccagaacagaagccctctccttaggcagaacatccaccccaggtcctgctcaatccacaatatcaccagaaatctccacggaaaccatcactagaatttctactcccctcaccacgacaggatcagcagaaatgaccatcacccccaaaacaggtcattctggggcatcctcacaaggtacctttaccttggacacatcaagcagagcctcctggccaggaactcactcagctgcaactcacagatctccacactcagggatgaccactcctatgagcagaggtcctgaggatgtgtcatggccaagccgcccatcagtggaaaaaactagccctccatcttccctggtgtctttatctgcagtaacctcaccttcgccactttattccacaccatctgagagtagccactcatctcctctccgggtgacttctcttttcacccctgtcatgatgaagaccacagacatgttggacacaagcttggaacctgtgaccacttcacctcccagtatgaatatcacctcagatgagagtctggccacttctaaagccaccatggagacagaggcaattcagctttcagaaaacacagctgtgactcagatgggcaccatcagcgctagacaagaattctattcctcttatccaggcctcccagagccatccaaagtgacatctccagtggtcacctcttccaccataaaagacattgtttctacaaccatacctgcttcctctgagataacaagaattgagatggagtcaacatccaccctgacccccacaccaagggagaccagcacctcccaggagatccactcagccacaaagccaagcactgttccttacaaggcactcactagtgccacgattgaggactccatgacacaagtcatgtcctctagcagaggacctagccctgatcagtccacaatgtcacaagacatatccactgaagtgatcaccaggctctctacctcccccatcaagacagaatctacagaaatgaccattaccacccaaacaggttctcctggggctacatcaaggggtacccttaccttggacacttcaacaacttttatgtcagggacccactcaactgcatctcaaggattttcacactcacagatgaccgctcttatgagtagaactcctggagatgtgccatggctaagccatccctctgtggaagaagccagctctgcctctttctcactgtcttcacctgtcatgacctcatcttctcccgtttcttccacattaccagacagcatccactcttcttcgcttcctgtgacatcacttctcacctcagggctggtgaagaccacagagctgttgggcacaagctcagaacctgaaaccagttcacccccaaatttgagcagcacctcagctgaaatactggccatcactgaagtcactacagatacagagaaactggagatgaccaatgtggtaacctcaggttatacacatgaatctccttcctctgtcctagctgactcagtgacaacaaaggccacatcttcaatgggtatcacctaccccacaggagatacaaatgttctcacatcaacccctgccttctctgacaccagtaggattcaaacaaagtcaaagctctcactgactcctgggttgatggagaccagcatctctgaagagaccagctctgccacagaaaaaagcactgtcctttctagtgtgcccactggtgctactactgaggtctccaggacagaagccatctcttctagcagaacatccatcccaggccctgctcaatccacaatgtcatcagacacctccatggaaaccatcactagaatttctacccccctcacaaggaaagaatcaacagacatggccatcacccccaaaacaggtccttctggggctacctcgcagggtacctttaccttggactcatcaagcacagcctcctggccaggaactcactcagctacaactcagagatttccacagtcagtggtgacaactcctatgagcagaggtcctgaggatgtgtcatggccaagcccgctgtctgtggaaaaaaacagccctccatcttccctggtatcttcatcttcagtaacctcaccttcgccactttattccacaccatctgggagtagccactcctctcctgtccctgtcacttctcttttcacctctatcatgatgaaggccacagacatgttggatgcaagtttggaacctgagaccacttcagctcccaatatgaatatcacctcagatgagagtctggccgcttctaaagccaccacggagacagaggcaattcacgtttttgaaaatacagcagcgtcccatgtggaaaccaccagtgctacagaggaactctattcctcttccccaggcttctcagagccaacaaaagtgatatctccagtggtcacctcttcctctataagagacaacatggtttccacaacaatgcctggctcctctggcattacaaggattgagatagagtcaatgtcatctctgacccctggactgagggagaccagaacctcccaggacatcacctcatccacagagacaagcactgtcctttacaagatgccctctggtgccactcctgaggtctccaggacagaagttatgccctctagcagaacatccattcctggccctgctcagtccacaatgtcactagacatctccgatgaagttgtcaccaggctgtctacctctcccatcatgacagaatctgcagaaataaccatcaccacccaaacaggttattctctggctacatcccaggttacccttcccttgggcacctcaatgacctttttgtcagggacccactcaactatgtctcaaggactttcacactcagagatgaccaatcttatgagcaggggtcctgaaagtctgtcatggacgagccctcgctttgtggaaacaactagatcttcctcttctctgacatcattacctctcacgacctcactttctcctgtgtcctccacattactagacagtagcccctcctctcctcttcctgtgacttcacttatcctcccaggcctggtgaagactacagaagtgttggatacaagctcagagcctaaaaccagttcatctccaaatttgagcagcacctcagttgaaataccggccacctctgaaatcatgacagatacagagaaaattcatccttcctcaaacacagcggtggccaaagtgaggacctccagttctgttcatgaatctcattcctctgtcctagctgactcagaaacaaccataaccataccttcaatgggtatcacctccgctgtggacgataccactgttttcacatcaaatcctgccttctctgagactaggaggattccgacagagccaacattctcattgactcctggattcagggagactagcacctctgaagagaccacctcaatcacagaaacaagtgcagtcctttatggagtgcccactagtgctactactgaagtctccatgacagaaatcatgtcctctaatagaatacacatccctgactctgatcagtccacgatgtctccagacatcatcactgaagtgatcaccaggctctcttcctcatccatgatgtcagaatcaacacaaatgaccatcaccacccaaaaaagttctcctggggctacagcacagagtactcttaccttggccacaacaacagcccccttggcaaggacccactcaactgttcctcctagatttttacactcagagatgacaactcttatgagtaggagtcctgaaaatccatcatggaagagctctctctttgtggaaaaaactagctcttcatcttctctgttgtccttacctgtcacgacctcaccttctgtttcttccacattaccgcagagtatcccttcctcctctttttctgtgacttcactcctcaccccaggcatggtgaagactacagacacaagcacagaacctggaaccagtttatctccaaatctgagtggcacctcagttgaaatactggctgcctctgaagtcaccacagatacagagaaaattcatccttcttcaagcatggcagtgaccaatgtgggaaccaccagttctggacatgaactatattcctctgtttcaatccactcggagccatccaaggctacatacccagtgggtactccctcttccatggctgaaacctctatttccacatcaatgcctgctaattttgagaccacaggatttgaggctgagccattttctcatttgacttctggatttaggaagacaaacatgtccctggacaccagctcagtcacaccaacaaatacaccttcttctcctgggtccactcaccttttacagagttccaagactgatttcacctcttctgcaaaaacatcatccccagactggcctccagcctcacagtatactgaaattccagtggacataatcaccccctttaatgcttctccatctattacggagtccactgggataacctccttcccagaatccaggtttactatgtctgtaacagaaagtactcatcatctgagtacagatttgctgccttcagctgagactatttccactggcacagtgatgccttctctatcagaggccatgacttcatttgccaccactggagttccacgagccatctcaggttcaggtagtccattctctaggacagagtcaggccctggggatgctactctgtccaccattgcagagagcctgccttcatccactcctgtgccattctcctcttcaaccttcactaccactgattcttcaaccatcccagccctccatgagataacttcctcttcagctaccccatatagagtggacaccagtcttgggacagagagcagcactactgaaggacgcttggttatggtcagtactttggacacttcaagccaaccaggcaggacatcttcatcacccattttggataccagaatgacagagagcgttgagctgggaacagtgacaagtgcttatcaagttccttcactctcaacacggttgacaagaactgatggcattatggaacacatcacaaaaatacccaatgaagcagcacacagaggtaccataagaccagtcaaaggccctcagacatccacttcgcctgccagtcctaaaggactacacacaggagggacaaaaagaatggagaccaccaccacagctctgaagaccaccaccacagctctgaagaccacttccagagccaccttgaccaccagtgtctatactcccactttgggaacactgactcccctcaatgcatcaatgcaaatggccagcacaatccccacagaaatgatgatcacaaccccatatgttttccctgatgttccagaaacgacatcctcattggctaccagcctgggagcagaaaccagcacagctcttcccaggacaaccccatctgttttcaatagagaatcagagaccacagcctcactggtctctcgttctggggcagagagaagtccggttattcaaactctagatgtttcttctagtgagccagatacaacagcttcatgggttatccatcctgcagagaccatcccaactgtttccaagacaacccccaattttttccacagtgaattagacactgtatcttccacagccaccagtcatggggcagacgtcagctcagccattccaacaaatatctcacctagtgaactagatgcactgaccccactggtcactatttcggggacagatactagtacaacattcccaacactgactaagtccccacatgaaacagagacaagaaccacatggctcactcatcctgcagagaccagctcaactattcccagaacaatccccaatttttctcatcatgaatcagatgccacaccttcaatagccaccagtcctggggcagaaaccagttcagctattccaattatgactgtctcacctggtgcagaagatctggtgacctcacaggtcactagttctgggacagacagaaatatgactattccaactttgactctttctcctggtgaaccaaagacgatagcctcattagtcacccatcctgaagcacagacaagttcggccattccaacttcaactatctcgcctgctgtatcacggttggtgacctcaatggtcaccagtttggcggcaaagacaagtacaactaatcgagctctgacaaactcccctggtgaaccagctacaacagtttcattggtcacgcatcctgcacagaccagcccaacagttccctggacaacttccatttttttccatagtaaatcagacaccacaccttcaatgaccaccagtcatggggcagaatccagttcagctgttccaactccaactgtttcaactgaggtaccaggagtagtgacccctttggtcaccagttctagggcagtgatcagtacaactattccaattctgactctttctcctggtgaaccagagaccacaccttcaatggccaccagtcatggggaagaagccagttctgctattccaactccaactgtttcacctggggtaccaggagtggtgacctctctggtcactagttctagggcagtgactagtacaactattccaattctgactttttctcttggtgaaccagagaccacaccttcaatggccaccagtcatgggacagaagctggctcagctgttccaactgttttacctgaggtaccaggaatggtgacctctctggttgctagttctagggcagtaaccagtacaactcttccaactctgactctttctcctggtgaaccagagaccacaccttcaatggccaccagtcatggggcagaagccagctcaactgttccaactgtttcacctgaggtaccaggagtggtgacctctctggtcactagttctagtggagtaaacagtacaagtattccaactctgattctttctcctggtgaactagaaaccacaccttcaatggccaccagtcatggggcagaagccagctcagctgttccaactccaactgtttcacctggggtatcaggagtggtgacccctctggtcactagttccagggcagtgaccagtacaactattccaattctaactctttcttctagtgagccagagaccacaccttcaatggccaccagtcatggggtagaagccagctcagctgttctaactgtttcacctgaggtaccaggaatggtgacctctctggtcactagttctagagcagtaaccagtacaactattccaactctgactatttcttctgatgaaccagagaccacaacttcattggtcacccattctgaggcaaagatgatttcagccattccaactttagctgtctcccctactgtacaagggctggtgacttcactggtcactagttctgggtcagagaccagtgcgttttcaaatctaactgttgcctcaagtcaaccagagaccatagactcatgggtcgctcatcctgggacagaagcaagttctgttgttccaactttgactgtctccactggtgagccgtttacaaatatctcattggtcacccatcctgcagagagtagctcaactcttcccaggacaacctcaaggttttcccacagtgaattagacactatgccttctacagtcaccagtcctgaggcagaatccagctcagccatttcaacaactatttcacctggtataccaggtgtgctgacatcactggtcactagctctgggagagacatcagtgcaacttttccaacagtgcctgagtccccacatgaatcagaggcaacagcctcatgggttactcatcctgcagtcaccagcacaacagttcccaggacaacccctaattattctcatagtgaaccagacaccacaccatcaatagccaccagtcctggggcagaagccacttcagattttccaacaataactgtctcacctgatgtaccagatatggtaacctcacaggtcactagttctgggacagacaccagtataactattccaactctgactctttcttctggtgagccagagaccacaacctcatttatcacctattctgagacacacacaagttcagccattccaactctccctgtctcccctggtgcatcaaagatgctgacctcactggtcatcagttctgggacagacagcactacaactttcccaacactgacggagaccccatatgaaccagagacaacagccatacagctcattcatcctgcagagaccaacacaatggttcccaggacaactcccaagttttcccatagtaagtcagacaccacactcccagtagccatcaccagtcctgggccagaagccagttcagctgtttcaacgacaactatctcacctgatatgtcagatctggtgacctcactggtccctagttctgggacagacaccagtacaaccttcccaacattgagtgagaccccatatgaaccagagactacagccacgtggctcactcatcctgcagaaaccagcacaacggtttctgggacaattcccaacttttcccataggggatcagacactgcaccctcaatggtcaccagtcctggagtagacacgaggtcaggtgttccaactacaaccatcccacccagtataccaggggtagtgacctcacaggtcactagttctgcaacagacactagtacagctattccaactttgactccttctcctggtgaaccagagaccacagcctcatcagctacccatcctgggacacagactggcttcactgttccaattcggactgttccctctagtgagccagatacaatggcttcctgggtcactcatcctccacagaccagcacacctgtttccagaacaacctccagtttttcccatagtagtccagatgccacacctgtaatggccaccagtcctaggacagaagccagttcagctgtactgacaacaatctcacctggtgcaccagagatggtgacttcacagatcactagttctggggcagcaaccagtacaactgttccaactttgactcattctcctggtatgccagagaccacagccttattgagcacccatcccagaacagagacaagtaaaacatttcctgcttcaactgtgtttcctcaagtatcagagaccacagcctcactcaccattagacctggtgcagagactagcacagctctcccaactcagacaacatcctctctcttcaccctacttgtaactggaaccagcagagttgatctaagtccaactgcttcacctggtgtttctgcaaaaacagccccactttccacccatccagggacagaaaccagcacaatgattccaacttcaactctttcccttggtttactagagactacaggcttactggccaccagctcttcagcagagaccagcacgagtactctaactctgactgtttcccctgctgtctctgggctttccagtgcctctataacaactgataagccccaaactgtgacctcctggaacacagaaacctcaccatctgtaacttcagttggacccccagaattttccaggactgtcacaggcaccactatgaccttgataccatcagagatgccaacaccacctaaaaccagtcatggagaaggagtgagtccaaccactatcttgagaactacaatggttgaagccactaatttagctaccacaggttccagtcccactgtggccaagacaacaaccaccttcaatacactggctggaagcctctttactcctctgaccacacctgggatgtccaccttggcctctgagagtgtgacctcaagaacaagttataaccatcggtcctggatctccaccaccagcagttataaccgtcggtactggacccctgccaccagcactccagtgacttctacattctccccagggatttccacatcctccatccccagctccacagcagccacagtcccattcatggtgccattcaccctcaacttcaccatcaccaacctgcagtacgaggaggacatgcggcaccctggttccaggaagttcaacgccacagagagagaactgcagggtctgctcaaacccttgttcaggaatagcagtctggaatacctctattcaggctgcagactagcctcactcaggccagagaaggatagctcagccacggcagtggatgccatctgcacacatcgccctgaccctgaagacctcggactggacagagagcgactgtactgggagctgagcaatctgacaaatggcatccaggagctgggcccctacaccctggaccggaacagtctctatgtcaatggtttcacccatcgaagctctatgcccaccaccagcactcctgggacctccacagtggatgtgggaacctcagggactccatcctccagccccagccccacgactgctggccctctcctgatgccgttcaccctcaacttcaccatcaccaacctgcagtacgaggaggacatgcgtcgcactggctccaggaagttcaacaccatggagagtgtcctgcagggtctgctcaagcccttgttcaagaacaccagtgttggccctctgtactctggctgcagattgaccttgctcaggcccgagaaagatggggcagccactggagtggatgccatctgcacccaccgccttgaccccaaaagccctggactcaacagggagcagctgtactgggagctaagcaaactgaccaatgacattgaagagctgggcccctacaccctggacaggaacagtctctatgtcaatggtttcacccatcagagctctgtgtccaccaccagcactcctgggacctccacagtggatctcagaacctcagggactccatcctccctctccagccccacaattatggctgctggccctctcctggtaccattcaccctcaacttcaccatcaccaacctgcagtatggggaggacatgggtcaccctggctccaggaagttcaacaccacagagagggtcctgcagggtctgcttggtcccatattcaagaacaccagtgttggccctctgtactctggctgcagactgacctctctcaggtctgagaaggatggagcagccactggagtggatgccatctgcatccatcatcttgaccccaaaagccctggactcaacagagagcggctgtactgggagctgagccaactgaccaatggcatcaaagagctgggcccctacaccctggacaggaacagtctctatgtcaatggtttcacccatcggacctctgtgcccaccagcagcactcctgggacctccacagtggaccttggaacctcagggactccattctccctcccaagccccgcaactgctggccctctcctggtgctgttcaccctcaacttcaccatcaccaacctgaagtatgaggaggacatgcatcgccctggctccaggaagttcaacaccactgagagggtcctgcagactctgcttggtcctatgttcaagaacaccagtgttggccttctgtactctggctgcagactgaccttgctcaggtccgagaaggatggagcagccactggagtggatgccatctgcacccaccgtcttgaccccaaaagccctggagtggacagggagcagctatactgggagctgagccagctgaccaatggcatcaaagagctgggcccctacaccctggacaggaacagtctctatgtcaatggtttcacccattggatccctgtgcccaccagcagcactcctgggacctccacagtggaccttgggtcagggactccatcctccctccccagccccacaactgctggccctctcctggtgccgttcaccctcaacttcaccatcaccaacctgaagtacgaggaggacatgcattgccctggctccaggaagttcaacaccacagagagagtcctgcagagtctgcttggtcccatgttcaagaacaccagtgttggccctctgtactctggctgcagactgaccttgctcaggtccgagaaggatggagcagccactggagtggatgccatctgcacccaccgtcttgaccccaaaagccctggagtggacagggagcagctatactgggagctgagccagctgaccaatggcatcaaagagctgggtccctacaccctggacagaaacagtctctatgtcaatggtttcacccatcagacctctgcgcccaacaccagcactcctgggacctccacagtggaccttgggacctcagggactccatcctccctccccagccctacatctgctggccctctcctggtgccattcaccctcaacttcaccatcaccaacctgcagtacgaggaggacatgcatcacccaggctccaggaagttcaacaccacggagcgggtcctgcagggtctgcttggtcccatgttcaagaacaccagtgtcggccttctgtactctggctgcagactgaccttgctcaggcctgagaagaatggggcagccactggaatggatgccatctgcagccaccgtcttgaccccaaaagccctggactcaacagagagcagctgtactgggagctgagccagctgacccatggcatcaaagagctgggcccctacaccctggacaggaacagtctctatgtcaatggtttcacccatcggagctctgtggcccccaccagcactcctgggacctccacagtggaccttgggacctcagggactccatcctccctccccagccccacaacagctgttcctctcctggtgccgttcaccctcaactttaccatcaccaatctgcagtatggggaggacatgcgtcaccctggctccaggaagttcaacaccacagagagggtcctgcagggtctgcttggtcccttgttcaagaactccagtgtcggccctctgtactctggctgcagactgatctctctcaggtctgagaaggatggggcagccactggagtggatgccatctgcacccaccaccttaaccctcaaagccctggactggacagggagcagctgtactggcagctgagccagatgaccaatggcatcaaagagctgggcccctacaccctggaccggaacagtctctacgtcaatggtttcacccatcggagctctgggctcaccaccagcactccttggacttccacagttgaccttggaacctcagggactccatcccccgtccccagccccacaaccaccggccctctcctggtgccattcacactcaacttcaccatcactaacctacagtatgaggagaacatgggtcaccctggctccaggaagttcaacatcacggagagtgttctgcagggtctgctcaagcccttgttcaagagcaccagtgttggccctctgtattctggctgcagactgaccttgctcaggcctgagaaggatggagtagccaccagagtggacgccatctgcacccaccgccctgaccccaaaatccctgggctagacagacagcagctatactgggagctgagccagctgacccacagcatcactgagctgggaccctacaccctggatagggacagtctctatgtcaatggtttcacccagcggagctctgtgcccaccaccagcactcctgggactttcacagtacagccggaaacctctgagactccatcatccctccctggccccacagccactggccctgtcctgctgccattcaccctcaattttaccatcactaacctgcagtatgaggaggacatgcgtcgccctggctccaggaagttcaacaccacggagagggtccttcagggtctgcttatgcccttgttcaagaacaccagtgtcagctctctgtactctggttgcagactgaccttgctcaggcctgagaaggatggggcagccaccagagtggatgctgtctgcacccatcgtcctgaccccaaaagccctggactggacagagagcggctgtactggaagctgagccagctgacccacggcatcactgagctgggcccctacaccctggacaggcacagtctctatgtcaatggtttcacccatcagagctctatgacgaccaccagaactcctgatacctccacaatgcacctggcaacctcgagaactccagcctccctgtctggacccatgaccgccagccctctcctggtgctattcacaattaacttcaccatcactaacctgcggtatgaggagaacatgcatcaccctggctctagaaagtttaacaccacggagagagtccttcagggtctgctcaggcctgtgttcaagaacaccagtgttggccctctgtactctggctgcagactgaccttgctcaggcccaagaaggatggggcagccaccaaagtggatgccatctgcacctaccgccctgatcccaaaagccctggactggacagagagcagctatactgggagctgagccagctgacccacagcatcactgagctgggcccctacaccctggacagggacagtctctatgtcaatggtttcacacagcggagctctgtgcccaccactagcattcctgggacccccacagtggacctgggaacatctgggactccagtttctaaacctggtccctcggctgccagccctctcctggtgctattcactctcaacttcaccatcaccaacctgcggtatgaggagaacatgcagcaccctggctccaggaagttcaacaccacggagagggtccttcagggcctgctcaggtccctgttcaagagcaccagtgttggccctctgtactctggctgcagactgactttgctcaggcctgaaaaggatgggacagccactggagtggatgccatctgcacccaccaccctgaccccaaaagccctaggctggacagagagcagctgtattgggagctgagccagctgacccacaatatcactgagctgggcccctatgccctggacaacgacagcctctttgtcaatggtttcactcatcggagctctgtgtccaccaccagcactcctgggacccccacagtgtatctgggagcatctaagactccagcctcgatatttggcccttcagctgccagccatctcctgatactattcaccctcaacttcaccatcactaacctgcggtatgaggagaacatgtggcctggctccaggaagttcaacactacagagagggtccttcagggcctgctaaggcccttgttcaagaacaccagtgttggccctctgtactctggctgcaggctgaccttgctcaggccagagaaagatggggaagccaccggagtggatgccatctgcacccaccgccctgaccccacaggccctgggctggacagagagcagctgtatttggagctgagccagctgacccacagcatcactgagctgggcccctacacactggacagggacagtctctatgtcaatggtttcacccatcggagctctgtacccaccaccagcaccggggtggtcagcgaggagccattcacactgaacttcaccatcaacaacctgcgctacatggcggacatgggccaacccggctccctcaagttcaacatcacagacaacgtcatgcagcacctgctcagtcctttgttccagaggagcagcctgggtgcacggtacacaggctgcagggtcatcgcactaaggtctgtgaagaacggtgctgagacacgggtggacctcctctgcacctacctgcagcccctcagcggcccaggtctgcctatcaagcaggtgttccatgagctgagccagcagacccatggcatcacccggctgggcccctactctctggacaaagacagcctctaccttaacggttacaatgaacctggtccagatgagcctcctacaactcccaagccagccaccacattcctgcctcctctgtcagaagccacaacagccatggggtaccacctgaagaccctcacactcaacttcaccatctccaatctccagtattcaccagatatgggcaagggctcagctacattcaactccaccgagggggtccttcagcacctgctcagacccttgttccagaagagcagcatgggccccttctacttgggttgccaactgatctccctcaggcctgagaaggatggggcagccactggtgtggacaccacctgcacctaccaccctgaccctgtgggccccgggctggacatacagcagctttactgggagctgagtcagctgacccatggtgtcacccaactgggcttctatgtcctggacagggatagcctcttcatcaatggctatgcaccccagaatttatcaatccggggcgagtaccagataaatttccacattgtcaactggaacctcagtaatccagaccccacatcctcagagtacatcaccctgctgagggacatccaggacaaggtcaccacactctacaaaggcagtcaactacatgacacattccgcttctgcctggtcaccaacttgacgatggactccgtgttggtcactgtcaaggcattgttctcctccaatttggaccccagcctggtggagcaagtctttctagataagaccctgaatgcctcattccattggctgggctccacctaccagttggtggacatccatgtgacagaaatggagtcatcagtttatcaaccaacaagcagctccagcacccagcacttctacctgaatttcaccatcaccaacctaccatattcccaggacaaagcccagccaggcaccaccaattaccagaggaacaaaaggaatattgaggatgcgctcaaccaactcttccgaaacagcagcatcaagagttatttttctgactgtcaagtttcaacattcaggtctgtccccaacaggcaccacaccggggtggactccctgtgtaacttctcgccactggctcggagagtagacagagttgccatctatgaggaatttctgcggatgacccggaatggtacccagctgcagaacttcaccctggacaggagcagtgtccttgtggatgggtattctcccaacagaaatgagcccttaactgggaattctgaccttcccttctgggctgtcatcctcatcggcttggcaggactcctgggagtcatcacatgcctgatctgcggtgtcctggtgaccacccgccggcggaagaaggaaggagaatacaacgtccagcaacagtgcccaggctactaccagtcacacctagacctggaggatctgcaatgactggaacttgccggtgcctggggtgcctttcccccagccagggtccaaagaagcttggctggggcagaaataaaccatattggtcgga

SEQ ID NO: 138 - protein, 518 aa, synthetic construct
  REGION 1..518: note = Bispecific
EIVMTQTPATLSVSAGERVTITCKASQSVSNDVTWYQQKPGQAPRLLIYSASNRYSGVPARFSGSGYGTEFTFTISSVQSEDFAVYFCQQDYSSFGQGTKLEIKRTVAAPSVFIFPPSDEQLKSGTASVVCLLNNFYPREAKVQWKVDNALQSGNSQESVTEQDSKDSTYSLSSTLTLSKADYEKHKVYACEVTHQGLSSPVTKSFNRGECGGGGSGGGGSQVQLVQSGGGLTLSKADYEKHKVYACEVTHQGLSSPVTKSFNRGECGGGGSGGGGSQVQLVQSGGGVVQPGRSLRLSCKASGYTFTRYTMHWVRQAPGKCLEWIGYINPSRGYTNYNQKFKDRFTISRDNSKNTAFLQMDSLRPEDTGVYFCARYYDDHYCLDYWGQGTPVTVSSGGGGSGGGGSGGGGSDIQMTQSPSSLSASVGDRVTITCSASSSVSYMNWYQQTPGKAPKRWIYDTSKLASGVPSRFSGSGSGTDYTFTISSLQPEDIATYYCQQWSSNPFTFGCGTKLQITR

SEQ ID NO: 139 - protein, 114 aa, synthetic construct
  REGION 1..114: note = MUC16c114-N3
NFSPLARRVDRVAIYEEFLRMTRNGTQLQAFTLDRSSVLVDGYSPNRNEPLTGNSDLPFWAVILIGLAGLLGLITCLICGVLVTTRRRKKEGEYNVQQQCPGYYQSHLDLEDLQ

SEQ ID NO: 140 - DNA, 366 bp, synthetic construct
  misc_feature 1..366: note = 10C6 VH NUCLEIC ACID
  source 1..366: mol_type = other DNA
caggtaactctgaaagagtctggccctgggatattgcagccctcccagaccctcagtctgacttgttctttctctgggttttcactgaacactcttggtatgggtgtaggctggattcggcagccttcagggaagggtctggagtggctggcacacatttggtgggatgatgataagtactataacccagccctgaagagtcggctcacaatctccaaggattcctccaaaaaccaggttttcctcaagatcgccaatgtggacactgcagatattgccacatactactgttctcgaatcgggacagctcaggctacggatgctctggactactggggtcaaggaacctcagtcaccgtctcctca

SEQ ID NO: 141 - DNA, 330 bp, synthetic construct
  misc_feature 1..330: note = 10C6 VL NUCLEIC ACID
  source 1..330: mol_type = other DNA
gacattgtgctgacacagtctcctgcttccttagctgtatctctggggcagagggccaccatctcatacagggccagcaaaagtgtcagtacatctggctatagttatatgcactggaaccaacagaaaccaggacagccacccagactcctcatctatcttgtatccaacctagaatctggggtccctgccaggttcagtggcagtgggtctgggacagacttcaccctcaacatccatcctgtggaggaggaggatgctgcaacctattactgtcagcacattagggagcttacacgttcggaggggggaccaagctggaaataaaac

SEQ ID NO: 142 - DNA, 369 bp, synthetic construct
  misc_feature 1..369: note = 7B12 VH NUCLEIC ACID
  source 1..369: mol_type = other DNA
caggttactctgaaagagtctggccctgggatattgcagccctcccagaccctcagtctgacttgttctttctctgggttttcactgagcactgttggtatgggtgtaggctggagtcgtcagccctcagggaagggtctggagtggctggcacacatctggtgggatgatgaagataagtattataatccagccctgaagagtcggctcacaatctccaaggatacctccaaaaaccaggtcttcctcaagatcgccaatgtggacactgcagatagtgccacatactactgtactcgaatcgggacagctcaggctacggatgctttggactactggggtcaaggaacctcagtcaccgtctcctca

SEQ ID NO: 143 - DNA, 336 bp, synthetic construct
  misc_feature 1..336: note = 7B12 VL NUCLEIC ACID
  source 1..336: mol_type = other DNA
gatattgtgatgactcaggctgcaccctctgtatctgtcactcctggagagtcagtatccatctcctgcaggtctagtaagagtcttcggaaaagtaatggcaacacttacttgtattggttcctgcagaggccaggccagtctcctcagcgcctgatatattatatgtccaaccttgcctcaggagtcccagacaggttcagtggcagagggtcaggaactgatttcacactgagaatcagtagagtggaggctgaagatgtgggtgtttattactgtatgcaaagtctagaatatcctctcacgttcggaggggggactaagctaaaaataaaa

SEQ ID NO: 144 - DNA, 366 bp, synthetic construct
  misc_feature 1..366: note = 19C11 VH NUCLEIC ACID
  source 1..366: mol_type = other DNA
caggttaatctgaaagagtctggccctgggaaattgcagccctcccagaccctcagtctgacttgttctttctctgggttttcactgagcactcttggtatgggtgtaggttggattcgtcagtcttcagggaagggtctggagtggctggcacacatttggtgggatgatgataagtactataacccagccctgaagagtcggctcacaatctccagggctacctccaaaaaccaggttttcctcaagatcgtcaatgtgggcactgcagatactgccacatattactgtgctcgaatcgggacagctcaggctacggatgctttggactattggggtcagggaacctcagtcaccgtttcctca

SEQ ID NO: 145 - DNA, 336 bp, synthetic construct
  misc_feature 1..336: note = 19C11 VL NUCLEIC ACID
  source 1..336: mol_type = other DNA
gatattgtgatgactcaggctgcaccctctatccctgtcactcctggagagtcagtatccatctcctgcaggtctagtaagagtcttctgcatagtaatggcaacacttatttgtattggttcctgcagaggccaggccagtctcctcagcgcctgatatattatatgtccaaccttgcctcaggagtcccagacaggttcagtggcagagggtcaggaactgatttcacactgaaaatcagtagagtggaggctggggatgtgggtgtttattactgtatgcagggtctagagcatcctctcacgttcggaggggggaccaagctggaaataaaa

SEQ ID NO: 146 - DNA, 366 bp, synthetic construct
  misc_feature 1..366: note = 16C5 VH NUCLEIC ACID
  source 1..366: mol_type = other DNA
caggttactctgaaagagtctggccctggaatattgcagccctcccagaccctcagtctgacttgttctttctctgggttttcactgaacactcttggtatgggtgtaggctggattcgtcagccttcagggaagggtctggagtggctggcacacatttggtgggatgatgataagtactattacccagccctgaagagtcggctcacaatctccagggatacctccaaaaaccaggtattcctcaagatcgccaatgtggacactgcagatactgccacatactactgtgctcgaatcgggacagctcaggctacggatgctctggactactggggtcaaggaacctcagtcaccgtctcctca

SEQ ID NO: 147 - DNA, 327 bp, synthetic construct
  misc_feature 1..327: note = 16C5 VL NUCLEIC ACID
  source 1..327: mol_type = other DNA
gagctcgatatgacccagactccaccctccctgtctgcatctgtgggagaaactgtcaggattaggtgcctggccagtgaggacatttatagtggtatatcctggtatcaacagaagccagggaaacctcctacactcctgatctatggtgcatccaatttagaatctggggtcccaccacggttcagtggcagtggatctgggacagattacaccctcaccattggcggcgtgcaggctgaagatgctgccacctactactgtctaggcggttatagttatagtagtaccttgacttttggagctggcaccaatgtggaaatcaaa

SEQ ID NO: 148 - DNA, 369 bp, synthetic construct
  misc_feature 1..369: note = 18C6 VH NUCLEIC ACID
  source 1..369: mol_type = other DNA
caggttactctgaaagagtctggccctgggatattgcagccctcccagaccctcagtctgacttgttctttctctgggttttcactgagcactgttggtatgggtgtaggctggagtcgtcagccttcagggaagggtctggagtggctggcacacatttggtgggatgatgaggataagtattataacccagccctgaagagtcggctcacaatctccaaggatacctccaaaaaccaggtattcctcaagatcgccaatgtggacactgcagatactgccacatactactgtactcgaatcgggacagctcaggctacggatgctttggactactggggtcaaggaacctcagtcaccgtctcctca

SEQ ID NO: 149 - DNA, 336 bp, synthetic construct
  misc_feature 1..336: note = 18C6 VL NUCLEIC ACID
  source 1..336: mol_type = other DNA
gatattgtgatgactcaggctgcaccctctgtacctgtcactcctggagagtcagtatccatctcctgcaggtctagtaagagtcttctgcatagtaatggcaacacttacttgtattggttcctgcagaggccaggccagtctcctcagcgcctgatatattatatgtccaaccttgcctcaggagtcccagacaggttcagtggcagagggtcaggaactgatttcacactgagaatcagtagagtggaggctgaggatgtgggtgtttattactgtatgcaaagtctagaatatcctctcacgttcggaggggggaccaagctggaaataaaa

SEQ ID NO: 150 - protein, 14447 aa, Homo sapiens
  REGION 1..14447: note = Mature Human MUC16 amino acid sequence
DKTLASPTSSVVGRTTQSLGVMSSALPESTSRGMTHSEQRTSPSLSPQVNGTPSRNYPATSMVSGLSSPRTRTSSTEGNFTKEASTYTLTVETTSGPVTEKYTVPTETSTTEGDSTETPWDTRYIPVKITSPMKTFADSTASKENAPVSMTPAETTVTDSHTPGRTNPSFGTLYSSFLDLSPKGTPNSRGETSLELILSTTGYPFSSPEPGSAGHSRISTSAPLSSSASVLDNKISETSIFSGQSLTSPLSPGVPEARASTMPNSAIPFSMTLSNAETSAERVRSTISSLGTPSISTKQTAETILTFHAFAETMDIPSTHIAKTLASEWLGSPGTLGGTSTSALTTTSPSTTLVSEETNTHHSTSGKETEGTLNTSMTPLETSAPGEESEMTATLVPTLGFTTLDSKIRSPSQVSSSHPTRELRTTGSTSGRQSSSTAAHGSSDILRATTSSTSKASSWTSESTAQQFSEPQHTQWVETSPSMKTERPPASTSVAAPITTSVPSVVSGFTTLKTSSTKGIWLEETSADTLIGESTAGPTTHQFAVPTGISMTGGSSTRGSQGTTHLLTRATASSETSADLTLATNGVPVSVSPAVSKTAAGSSPPGGTKPSYTMVSSVIPETSSLQSSAFREGTSLGLTPLNTRHPFSSPEPDSAGHTKISTSIPLLSSASVLEDKVSATSTFSHHKATSSITTGTPEISTKTKPSSAVLSSMTLSNAATSPERVRNATSPLTHPSPSGEETAGSVLTLSTSAETTDSPNIHPTGTLTSESSESPSTLSLPSVSGVKTTFSSSTPSTHLFTSGEETEETSNPSVSQPETSVSRVRTTLASTSVPTPVFPTMDTWPTRSAQFSSSHLVSELRATSSTSVTNSTGSALPKISHLTGTATMSQTNRDTFNDSAAPQSTTWPETSPRFKTGLPSATTTVSTSATSLSATVMVSKFTSPATSSMEATSIREPSTTILTTETTNGPGSMAVASTNIPIGKGYITEGRLDTSHLPIGTTASSETSMDFTMAKESVSMSVSPSQSMDAAGSSTPGRTSQFVDTFSDDVYHLTSREITIPRDGTSSALTPQMTATHPPSPDPGSARSTWLGILSSSPSSPTPKVTMSSTFSTQRVTTSMIMDTVETSRWNMPNLPSTTSLTPSNIPTSGAIGKSTLVPLDTPSPATSLEASEGGLPTLSTYPESTNTPSIHLGAHASSESPSTIKLTMASVVKPGSYTPLTFPSIETHIHVSTARMAYSSGSSPEMTAPGETNTGSTWDPTTYITTTDPKDTSSAQVSTPHSVRTLRTTENHPKTESATPAAYSGSPKISSSPNLTSPATKAWTITDTTEHSTQLHYTKLAEKSSGFETQSAPGPVSVVIPTSPTIGSSTLELTSDVPGEPLVLAPSEQTTITLPMATWLSTSLTEEMASTDLDISSPSSPMSTFAIFPPMSTPSHELSKSEADTSAIRNTDSTTLDQHLGIRSLGRTGDLTTVPITPLTTTWTSVIEHSTQAQDTLSATMSPTHVTQSLKDQTSIPASASPSHLTEVYPELGTQGRSSSEATTFWKPSTDTLSREIETGPTNIQSTPPMDNTTTGSSSSGVTLGIAHLPIGTSSPAETSTNMALERRSSTATVSMAGTMGLLVTSAPGRSISQSLGRVSSVLSESTTEGVTDSSKGSSPRLNTQGNTALSSSLEPSYAEGSQMSTSIPLTSSPTTPDVEFIGGSTFWTKEVTTVMTSDISKSSARTESSSATLMSTALGSTENTGKEKLRTASMDLPSPTPSMEVTPWISLTLSNAPNTTDSLDLSHGVHTSSAGTLATDRSLNTGVTRASRLENGSDTSSKSLSMGNSTHTSMTYTEKSEVSSSIHPRPETSAPGAETTLTSTPGNRAISLTLPFSSIPVEEVISTGITSGPDINSAPMTHSPITPPTIVWTSTGTIEQSTQPLHAVSSEKVSVQTQSTPYVNSVAVSASPTHENSVSSGSSTSSPYSSASLESLDSTISRRNAITSWLWDLTTSLPTTTWPSTSLSEALSSGHSGVSNPSSTTTEFPLFSAASTSAAKQRNPETETHGPQNTAASTLNTDASSVTGLSETPVGASISSEVPLPMAITSRSDVSGLTSESTANPSLGTASSAGTKLTRTISLPTSESLVSFRMNKDPWTVSIPLGSHPTTNTETSIPVNSAGPPGLSTVASDVIDTPSDGAESIPTVSFSPSPDTEVTTISHFPEKTTHSFRTISSLTHELTSRVTPIPGDWMSSAMSTKPTGASPSITLGERRTITSAAPTTSPIVLTASFTETSTVSLDNETTVKTSDILDARKTNELPSDSSSSSDLINTSIASSTMDVTKTASISPTSISGMTASSSPSLFSSDRPQVPTSTTETNTATSPSVSSNTYSLDGGSNVGGTPSTLPPFTITHPVETSSALLAWSRPVRTFSTMVSTDTASGENPTSSNSVVTSVPAPGTWTSVGSTTDLPAMGFLKTSPAGEAHSLLASTIEPATAFTPHLSAAVVTGSSATSEASLLTTSESKAIHSSPQTPTTPTSGANWETSATPESLLVVTETSDTTLTSKILVTDTILFSTVSTPPSKFPSTGTLSGASFPTLLPDTPAIPLTATEPTSSLATSFDSTPLVTIASDSLGTVPETTLTMSETSNGDALVLKTVSNPDRSIPGITIQGVTESPLHPSSTSPSKIVAPRNTTYEGSITVALSTLPAGTTGSLVFSQSSENSETTALVDSSAGLERASVMPLTTGSQGMASSGGIRSGSTHSTGTKTFSSLPLTMNPGEVTAMSEITTNRLTATQSTAPKGIPVKPTSAESGLLTPVSASSSPSKAFASLTTAPPTWGIPQSTLTFEFSEVPSLDTKSASLPTPGQSLNTIPDSDASTASSSLSKSPEKNPRARMMTSTKAISASSFQSTGFTETPEGSASPSMAGHEPRVPTSGTGDPRYASESMSYPDPSKASSAMTSTSLASKLTTLFSTGQAARSGSSSSPISLSTEKETSFLSPTASTSRKTSLFLGPSMARQPNILVHLQTSALTLSPTSTLNMSQEEPPELTSSQTIAEEEGTTAETQTLTFTPSETPTSLLPVSSPTEPTARRKSSPETWASSISVPAKTSLVETTDGTLVTTIKMSSQAAQGNSTWPAPAEETGSSPAGTSPGSPEMSTTLKIMSSKEPSISPEIRSTVRNSPWKTPETTVPMETTVEPVTLQSTALGSGSTSISHLPTGTTSPTKSPTENMLATERVSLSPSPPEAWTNLYSGTPGGTRQSLATMSSVSLESPTARSITGTGQQSSPELVSKTTGMEFSMWHGSTGGTTGDTHVSLSTSSNILEDPVTSPNSVSSLTDKSKHKTETWVSTTAIPSTVLNNKIMAAEQQTSRSVDEAYSSTSSWSDQTSGSDITLGASPDVTNTLYITSTAQTTSLVSLPSGDQGITSLTNPSGGKTSSASSVTSPSIGLETLRANVSAVKSDIAPTAGHLSQTSSPAEVSILDVTTAPTPGISTTITTMGTNSISTTTPNPEVGMSTMDSTPATERRTTSTEHPSTWSSTAASDSWTVTDMTSNLKVARSPGTISTMHTTSFLASSTELDSMSTPHGRITVIGTSLVTPSSDASAVKTETSTSERTLSPSDTTASTPISTFSRVQRMSISVPDILSTSWTPSSTEAEDVPVSMVSTDHASTKTDPNTPLSTFLFDSLSTLDWDTGRSLSSATATTSAPQGATTPQELTLETMISPATSQLPFSIGHITSAVTPAAMARSSGVTFSRPDPTSKKAEQTSTQLPTTTSAHPGQVPRSAATTLDVIPHTAKTPDATFQRQGQTALTTEARATSDSWNEKEKSTPSAPWITEMMNSVSEDTIKEVTSSSSVLRTLNTLDINLESGTTSSPSWKSSPYERIAPSESTTDKEAIHPSTNTVETTGWVTSSEHASHSTIPAHSASSKLTSPVVTTSTREQAIVSMSTTTWPESTRARTEPNSFLTIELRDVSPYMDTSSTTQTSIISSPGSTAITKGPRTEITSSKRISSSFLAQSMRSSDSPSEAITRLSNFPAMTESGGMILAMQTSPPGATSLSAPTLDTSATASWTGTPLATTQRFTYSEKTTLFSKGPEDTSQPSPPSVEETSSSSSLVPIHATTSPSNILLTSQGHSPSSTPPVTSVFLSETSGLGKTTDMSRISLEPGTSLPPNLSSTAGEALSTYEASRDTKAIHHSADTAVTNMEATSSEYSPIPGHTKPSKATSPLVTSHIMGDITSSTSVFGSSETTEIETVSSVNQGLQERSTSQVASSATETSTVITHVSSGDATTHVTKTQATFSSGTSISSPHQFITSTNTFTDVSTNPSTSLIMTESSGVTITTQTGPTGAATQGPYLLDTSTMPYLTETPLAVTPDFMQSEKTTLISKGPKDVSWTSPPSVAETSYPSSLTPFLVTTIPPATSTLQGQHTSSPVSATSVLTSGLVKTTDMLNTSMEPVTNSPQNLNNPSNEILATLAATTDIETIHPSINKAVTNMGTASSAHVLHSTLPVSSEPSTATSPMVPASSMGDALASISIPGSETTDIEGEPTSSLTAGRKENSTLQEMNSTTESNIILSNVSVGAITEATKMEVPSFDATFIPTPAQSTKFPDIFSVASSRLSNSPPMTISTHMTTTQTGSSGATSKIPLALDTSTLETSAGTPSVVTEGFAHSKITTAMNNDVKDVSQTNPPFQDEASSPSSQAPVLVTTLPSSVAFTPQWHSTSSPVSMSSVLTSSLVKTAGKVDTSLETVTSSPQSMSNTLDDISVTSAATTDIETTHPSINTVVTNVGTTGSAFESHSTVSAYPEPSKVTSPNVTTSTMEDTTISRSIPKSSKTTRTETETTSSLTPKLRETSISQEITSSTETSTVPYKELTGATTEVSRTDVTSSSSTSFPGPDQSTVSLDISTETNTRLSTSPIMTESAEITITTQTGPHGATSQDTFTMDPSNTTPQAGIHSAMTHGFSQLDVTTLMSRIPQDVSWTSPPSVDKTSSPSSFLSSPAMTTPSLISSTLPEDKLSSPMTSLLTSGLVKITDILRTRLEPVTSSLPNFSSTSDKILATSKDSKDTKEIFPSINTEETNVKANNSGHESHSPALADSETPKATTQMVITTTVGDPAPSTSMPVHGSSETTNIKREPTYFLTPRLRETSTSQESSFPTDTSFLLSKVPTGTITEVSSTGVNSSSKISTPDHDKSTVPPDTFTGEIPRVFTSSIKTKSAEMTITTQASPPESASHSTLPLDTSTTLSQGGTHSTVTQGFPYSEVTTLMGMGPGNVSWMTTPPVEETSSVSSLMSSPAMTSPSPVSSTSPQSIPSSPLPVTALPTSVLVTTTDVLGTTSPESVTSSPPNLSSITHERPATYKDTAHTEAAMHHSTNTAVTNVGTSGSGHKSQSSVLADSETSKATPLMSTTSTLGDTSVSTSTPNISQTNQIQTEPTASLSPRLRESSTSEKTSSTTETNTAFSYVPTGAITQASRTEISSSRTSISDLDRPTIAPDISTGMITRLFTSPIMTKSAEMTVTTQTTTPGATSQGILPWDTSTTLFQGGTHSTVSQGFPHSEITTLRSRTPGDVSWMTTPPVEETSSGFSLMSPSMTSPSPVSSTSPESIPSSPLPVTALLTSVLVTTTNVLGTTSPEPVTSSPPNLSSPTQERLTTYKDTAHTEAMHASMHTNTAVANVGTSISGHESQSSVPADSHTSKATSPMGITFAMGDTSVSTSTPAFFETRIQTESTSSLIPGLRDTRTSEEINTVTETSTVLSEVPTTTTTEVSRTEVITSSRTTISGPDHSKMSPYISTETITRLSTFPFVTGSTEMAITNQTGPIGTISQATLTLDTSSTASWEGTHSPVTQRFPHSEETTTMSRSTKGVSWQSPPSVEETSSPSSPVPLPAITSHSSLYSAVSGSSPTSALPVTSLLTSGRRKTIDMLDTHSELVTSSLPSASSFSGEILTSEASTNTETIHFSENTAETNMGTTNSMHKLHSSVSIHSQPSGHTPPKVTGSMMEDAIVSTSTPGSPETKNVDRDSTSPLTPELKEDSTALVMNSTTESNTVFSSVSLDAATEVSRAEVTYYDPTFMPASAQSTKSPDISPEASSSHSNSPPLTISTHKTIATQTGPSGVTSLGQLTLDTSTIATSAGTPSARTQDFVDSETTSVMNNDLNDVLKTSPFSAEEANSLSSQAPLLVTTSPSPVTSTLQEHSTSSLVSVTSVPTPTLAKITDMDTNLEPVTRSPQNLRNTLATSEATTDTHTMHPSINTAVANVGTTSSPNEFYFTVSPDSDPYKATSAVVITSTSGDSIVSTSMPRSSAMKKIESETTFSLIFRLRETSTSQKIGSSSDTSTVFDKAFTAATTEVSRTELTSSSRTSIQGTEKPTMSPDTSTRSVTMLSTFAGLTKSEERTIATQTGPHRATSQGTLTWDTSITTSQAGTHSAMTHGFSQLDLSTLTSRVPEYISGTSPPSVEKTSSSSSLLSLPAITSPSPVPTTLPESRPSSPVHLTSLPTSGLVKTTDMLASVASLPPNLGSTSHKIPTTSEDIKDTEKMYPSTNIAVTNVGTTTSEKESYSSVPAYSEPPKVTSPMVTSFNIRDTIVSTSMPGSSEITRIEMESTFSLAHGLKGTSTSQDPIVSTEKSAVLHKLTTGATETSRTEVASSRRTSIPGPDHSTESPDISTEVIPSLPISLGITESSNMTIITRTGPPLGSTSQGTFTLDTPTTSSRAGTHSMATQEFPHSEMTTVMNKDPEILSWTIPPSIEKTSFSSSLMPSPAMTSPPVSSTLPKTIHTTPSPMTSLLTPSLVMTTDTLGTSPEPTTSSPPNLSSTSHEILTTDEDTTAIEAMHPSTSTAATNVETTSSGHGSQSSVLADSEKTKATAPMDTTSTMGHTTVSTSMSVSSETTKIKRESTYSLTPGLRETSISQNASFSTDTSIVLSEVPTGTTAEVSRTEVTSSGRTSIPGPSQSTVLPEISTRTMTRLFASPTMTESAEMTIPTQTGPSGSTSQDTLTLDTSTTKSQAKTHSTLTQRFPHSEMTTLMSRGPGDMSWQSSPSLENPSSLPSLLSLPATTSPPPISSTLPVTISSSPLPVTSLLTSSPVTTTDMLHTSPELVTSSPPKLSHTSDERLTTGKDTTNTEAVHPSTNTAASNVEIPSSGHESPSSALADSETSKATSPMFITSTQEDTTVAISTPHFLETSRIQKESISSLSPKLRETGSSVETSSAIETSAVLSEVSIGATTEISRTEVTSSSRTSISGSAESTMLPEISTTRKIIKFPTSPILAESSEMTIKTQTSPPGSTSESTFTLDTSTTPSLVITHSTMTQRLPHSEITTLVSRGAGDVPRPSSLPVEETSPPSSQLSLSAMISPSPVSSTLPASSHSSSASVTSLLTPGQVKTTEVLDASAEPETSSPPSLSSTSVEILATSEVTTDTEKIHPFSNTAVTKVGTSSSGHESPSSVLPDSETTKATSAMGTISIMGDTSVSTLTPALSNTRKIQSEPASSLTTRLRETSTSEETSLATEANTVLSKVSTGATTEVSRTEAISFSRTSMSGPEQSTMSQDISIGTIPRISASSVLTESAKMTITTQTGPSESTLESTLNLNTATTPSWVETHSIVIQGFPHPEMTTSMGRGPGGVSWPSPPFVKETSPPSSPLSLPAVTSPHPVSTTFLAHIPPSPLPVTSLLTSGPATTTDILGTSTEPGTSSSSSLSTTSHERLTTYKDTAHTEAVHPSTNTGGTNVATTSSGYKSQSSVLADSSPMCTTSTMGDTSVLTSTPAFLETRRIQTELASSLTPGLRESSGSEGTSSGTKMSTVLSKVPTGATTEISKEDVTSIPGPAQSTISPDISTRTVSWFSTSPVMTESAEITMNTHTSPLGATTQGTSTLDTSSTTSLTMTHSTISQGFSHSQMSTLMRRGPEDVSWMSPPLLEKTRPSFSLMSSPATTSPSPVSSTLPESISSSPLPVTSLLTSGLAKTTDMLHKSSEPVTNSPANLSSTSVEILATSEVTTDTEKTHPSSNRTVTDVGTSSSGHESTSFVLADSQTSKVTSPMVITSTMEDTSVSTSTPGFFETSRIQTEPTSSLTLGLRKTSSSEGTSLATEMSTVLSGVPTGATAEVSRTEVTSSSRTSISGFAQLTVSPETSTETITRLPTSSIMTESAEMMIKTQTDPPGSTPESTHTVDISTTPNWVETHSTVTQRFSHSEMTTLVSRSPGDMLWPSQSSVEETSSASSLLSLPATTSPSPVSSTLVEDFPSASLPVTSLLNPGLVITTDRMGISREPGTSSTSNLSSTSHERLTTLEDTVDTEDMQPSTHTAVTNVRTSISGHESQSSVLSDSETPKATSPMGTTYTMGETSVSISTSDFFETSRIQIEPTSSLTSGLRETSSSERISSATEGSTVLSEVPSGATTEVSRTEVISSRGTSMSGPDQFTISPDISTEAITRLSTSPIMTESAESAITIETGSPGATSEGTLTLDTSTTTFWSGTHSTASPGFSHSEMTTLMSRTPGDVPWPSLPSVEEASSVSSSLSSPAMTSTSFFSTLPESISSSPHPVTALLTLGPVKTTDMLRTSSEPETSSPPNLSSTSAEILATSEVTKDREKIHPSSNTPVVNVGTVIYKHLSPSSVLADLVTTKPTSPMATTSTLGNTSVSTSTPAFPETMMTQPTSSLTSGLREISTSQETSSATERSASLSGMPTGATTKVSRTEALSLGRTSTPGPAQSTISPEISTETITRISTPLTTTGSAEMTITPKTGHSGASSQGTFTLDTSSRASWPGTHSAATHRSPHSGMTTPMSRGPEDVSWPSRPSVEKTSPPSSLVSLSAVTSPSPLYSTPSESSHSSPLRVTSLFTPVMMKTTDMLDTSLEPVTTSPPSMNITSDESLATSKATMETEAIQLSENTAVTQMGTISARQEFYSSYPGLPEPSKVTSPVVTSSTIKDIVSTTIPASSEITRIEMESTSTLTPTPRETSTSQEIHSATKPSTVPYKALTSATIEDSMTQVMSSSRGPSPDQSTMSQDISTEVITRLSTSPIKTESTEMTITTQTGSPGATSRGTLTLDTSTTFMSGTHSTASQGFSHSQMTALMSRTPGDVPWLSHPSVEEASSASFSLSSPVMTSSSPVSSTLPDSIHSSSLPVTSLLTSGLVKTTELLGTSSEPETSSPPNLSSTSAEILAITEVTTDTEKLEMTNVVTSGYTHESPSSVLADSVTTKATSSMGITYPTGDTNVLTSTPAFSDTSRIQTKSKLSLTPGLMETSISEETSSATEKSTVLSSVPTGATTEVSRTEAISSSRTSIPGPAQSTMSSDTSMETITRISTPLTRKESTDMAITPKTGPSGATSQGTFTLDSSSTASWPGTHSATTQRFPQSVVTTPMSRGPEDVSWPSPLSVEKNSPPSSLVSSSSVTSPSPLYSTPSGSSHSSPVPVTSLFTSIMMKATDMLDASLEPETTSAPNMNITSDESLAASKATTETEAIHVFENTAASHVETTSATEELYSSSPGFSEPTKVISPVVTSSSIRDNMVSTTMPGSSGITRIEIESMSSLTPGLRETRTSQDITSSTETSTVLYKMPSGATPEVSRTEVMPSSRTSIPGPAQSTMSLDISDEVVTRLSTSPIMTESAEITITTQTGYSLATSQVTLPLGTSMTFLSGTHSTMSQGLSHSEMTNLMSRGPESLSWTSPRFVETTRSSSSLTSLPLTTSLSPVSSTLLDSSPSSPLPVTSLILPGLVKTTEVLDTSSEPKTSSSPNLSSTSVEIPATSEIMTDTEKIHPSSNTAVAKVRTSSSVHESHSSVLADSETTITIPSMGITSAVDDTTVFTSNPAFSETRRIPTEPTFSLTPGFRETSTSEETTSITETSAVLYGVPTSATTEVSMTEIMSSNRIHIPDSDQSTMSPDIITEVITRLSSSSMMSESTQMTITTQKSSPGATAQSTLTLATTTAPLARTHSTVPPRFLHSEMTTLMSRSPENPSWKSSLFVEKTSSSSSLLSLPVTTSPSVSSTLPQSIPSSSFSVTSLLTPGMVKTTDTSTEPGTSLSPNLSGTSVEILAASEVTTDTEKIHPSSSMAVTNVGTTSSGHELYSSVSIHSEPSKATYPVGTPSSMAETSISTSMPANFETTGFEAEPFSHLTSGFRKTNMSLDTSSVTPTNTPSSPGSTHLLQSSKTDFTSSAKTSSPDWPPASQYTEIPVDIITPFNASPSITESTGITSFPESRFTMSVTESTHHLSTDLLPSAETISTGTVMPSLSEAMTSFATTGVPRAISGSGSPFSRTESGPGDATLSTIAESLPSSTPVPFSSSTFTTTDSSTIPALHEITSSSATPYRVDTSLGTESSTTEGRLVMVSTLDTSSQPGRTSSSPILDTRMTESVELGTVTSAYQVPSLSTRLTRTDGIMEHITKIPNEAAHRGTIRPVKGPQTSTSPASPKGLHTGGTKRMETTTTALKTTTTALKTTSRATLTTSVYTPTLGTLTPLNASMQMASTIPTEMMITTPYVFPDVPETTSSLATSLGAETSTALPRTTPSVFNRESETTASLVSRSGAERSPVIQTLDVSSSEPDTTASWVIHPAETIPTVSKTTPNFFHSELDTVSSTATSHGADVSSAIPTNISPSELDALTPLVTISGTDTSTTFPTLTKSPHETETRTTWLTHPAETSSTIPRTIPNFSHHESDATPSIATSPGAETSSAIPIMTVSPGAEDLVTSQVTSSGTDRNMTIPTLTLSPGEPKTIASLVTHPEAQTSSAIPTSTISPAVSRLVTSMVTSLAAKTSTTNRALTNSPGEPATTVSLVTHPAQTSPTVPWTTSIFFHSKSDTTPSMTTSHGAESSSAVPTPTVSTEVPGVVTPLVTSSRAVISTTIPILTLSPGEPETTPSMATSHGEEASSAIPTPTVSPGVPGVVTSLVTSSRAVTSTTIPILTFSLGEPETTPSMATSHGTEAGSAVPTVLPEVPGMVTSLVASSRAVTSTTLPTLTLSPGEPETTPSMATSHGAEASSTVPTVSPEVPGVVTSLVTSSSGVNSTSIPTLILSPGELETTPSMATSHGAEASSAVPTPTVSPGVSGVVTPLVTSSRAVTSTTIPILTLSSSEPETTPSMATSHGVEASSAVLTVSPEVPGMVTSLVTSSRAVTSTTIPTLTISSDEPETTTSLVTHSEAKMISAIPTLAVSPTVQGLVTSLVTSSGSETSAFSNLTVASSQPETIDSWVAHPGTEASSVVPTLTVSTGEPFTNISLVTHPAESSSTLPRTTSRFSHSELDTMPSTVTSPEAESSSAISTTISPGIPGVLTSLVTSSGRDISATFPTVPESPHESEATASWVTHPAVTSTTVPRTTPNYSHSEPDTTPSIATSPGAEATSDFPTITVSPDVPDMVTSQVTSSGTDTSITIPTLTLSSGEPETTTSFITYSETHTSSAIPTLPVSPGASKMLTSLVISSGTDSTTTFPTLTETPYEPETTAIQLIHPAETNTMVPRTTPKFSHSKSDTTLPVAITSPGPEASSAVSTTTISPDMSDLVTSLVPSSGTDTSTTFPTLSETPYEPETTATWLTHPAETSTTVSGTIPNFSHRGSDTAPSMVTSPGVDTRSGVPTTTIPPSIPGVVTSQVTSSATDTSTAIPTLTPSPGEPETTASSATHPGTQTGFTVPIRTVPSSEPDTMASWVTHPPQTSTPVSRTTSSFSHSSPDATPVMATSPRTEASSAVLTTISPGAPEMVTSQITSSGAATSTTVPTLTHSPGMPETTALLSTHPRTETSKTFPASTVFPQVSETTASLTIRPGAETSTALPTQTTSSLFTLLVTGTSRVDLSPTASPGVSAKTAPLSTHPGTETSTMIPTSTLSLGLLETTGLLATSSSAETSTSTLTLTVSPAVSGLSSASITTDKPQTVTSWNTETSPSVTSVGPPEFSRTVTGTTMTLIPSEMPTPPKTSHGEGVSPTTILRTTMVEATNLATTGSSPTVAKTTTTFNTLAGSLFTPLTTPGMSTLASESVTSRTSYNHRSWISTTSSYNRRYWTPATSTPVTSTFSPGISTSSIPSSTAATVPFMVPFTLNFTITNLQYEEDMRHPGSRKFNATERELQGLLKPLFRNSSLEYLYSGCRLASLRPEKDSSATAVDAICTHRPDPEDLGLDRERLYWELSNLTNGIQELGPYTLDRNSLYVNGFTHRSSMPTTSTPGTSTVDVGTSGTPSSSPSPTTAGPLLMPFTLNFTITNLQYEEDMRRTGSRKFNTMESVLQGLLKPLFKNTSVGPLYSGCRLTLLRPEKDGAATGVDAICTHRLDPKSPGLNREQLYWELSKLTNDIEELGPYTLDRNSLYVNGFTHQSSVSTTSTPGTSTVDLRTSGTPSSLSSPTIMAAGPLLVPFTLNFTITNLQYGEDMGHPGSRKFNTTERVLQGLLGPIFKNTSVGPLYSGCRLTSLRSEKDGAATGVDAICIHHLDPKSPGLNRERLYWELSQLTNGIKELGPYTLDRNSLYVNGFTHRTSVPTSSTPGTSTVDLGTSGTPFSLPSPATAGPLLVLFTLNFTITNLKYEEDMHRPGSRKFNTTERVLQTLLGPMFKNTSVGLLYSGCRLTLLRSEKDGAATGVDAICTHRLDPKSPGVDREQLYWELSQLTNGIKELGPYTLDRNSLYVNGFTHWIPVPTSSTPGTSTVDLGSGTPSSLPSPTTAGPLLVPFTLNFTITNLKYEEDMHCPGSRKFNTTERVLQSLLGPMFKNTSVGPLYSGCRLTLLRSEKDGAATGVDAICTHRLDPKSPGVDREQLYWELSQLTNGIKELGPYTLDRNSLYVNGFTHQTSAPNTSTPGTSTVDLGTSGTPSSLPSPTSAGPLLVPFTLNFTITNLQYEEDMHHPGSRKFNTTERVLQGLLGPMFKNTSVGLLYSGCRLTLLRPEKNGAATGMDAICSHRLDPKSPGLNREQLYWELSQLTHGIKELGPYTLDRNSLYVNGFTHRSSVAPTSTPGTSTVDLGTSGTPSSLPSPTTAVPLLVPFTLNFTITNLQYGEDMRHPGSRKFNTTERVLQGLLGPLFKNSSVGPLYSGCRLISLRSEKDGAATGVDAICTHHLNPQSPGLDREQLYWQLSQMTNGIKELGPYTLDRNSLYVNGFTHRSSGLTTSTPWTSTVDLGTSGTPSPVPSPTTTGPLLVPFTLNFTITNLQYEENMGHPGSRKFNITESVLQGLLKPLFKSTSVGPLYSGCRLTLLRPEKDGVATRVDAICTHRPDPKIPGLDRQQLYWELSQLTHSITELGPYTLDRDSLYVNGFTQRSSVPTTSTPGTFTVQPETSETPSSLPGPTATGPVLLPFTLNFTITNLQYEEDMRRPGSRKFNTTERVLQGLLMPLFKNTSVSSLYSGCRLTLLRPEKDGAATRVDAVCTHRPDPKSPGLDRERLYWKLSQLTHGITELGPYTLDRHSLYVNGFTHQSSMTTTRTPDTSTMHLATSRTPASLSGPMTASPLLVLFTINFTITNLRYEENMHHPGSRKFNTTERVLQGLLRPVFKNTSVGPLYSGCRLTLLRPKKDGAATKVDAICTYRPDPKSPGLDREQLYWELSQLTHSITELGPYTLDRDSLYVNGFTQRSSVPTTSIPGTPTVDLGTSGTPVSKPGPSAASPLLVLFTLNFTITNLRYEENMQHPGSRKFNTTERVLQGLLRSLFKSTSVGPLYSGCRLTLLRPEKDGTATGVDAICTHHPDPKSPRLDREQLYWELSQLTHNITELGPYALDNDSLFVNGFTHRSSVSTTSTPGTPTVYLGASKTPASIFGPSAASHLLILFTLNFTITNLRYEENMWPGSRKFNTTERVLQGLLRPLFKNTSVGPLYSGCRLTLLRPEKDGEATGVDAICTHRPDPTGPGLDREQLYLELSQLTHSITELGPYTLDRDSLYVNGFTHRSSVPTTSTGVVSEEPFTLNFTINNLRYMADMGQPGSLKFNITDNVMQHLLSPLFQRSSLGARYTGCRVIALRSVKNGAETRVDLLCTYLQPLSGPGLPIKQVFHELSQQTHGITRLGPYSLDKDSLYLNGYNEPGPDEPPTTPKPATTFLPPLSEATTAMGYHLKTLTLNFTISNLQYSPDMGKGSATFNSTEGVLQHLLRPLFQKSSMGPFYLGCQLISLRPEKDGAATGVDTTCTYHPDPVGPGLDIQQLYWELSQLTHGVTQLGFYVLDRDSLFINGYAPQNLSIRGEYQINFHIVNWNLSNPDPTSSEYITLLRDIQDKVTTLYKGSQLHDTFRFCLVTNLTMDSVLVTVKALFSSNLDPSLVEQVFLDKTLNASFHWLGSTYQLVDIHVTEMESSVYQPTSSSSTQHFYLNFTITNLPYSQDKAQPGTTNYQRNKRNIEDALNQLFRNSSIKSYFSDCQVSTFRSVPNRHHTGVDSLCNFSPLARRVDRVAIYEEFLRMTRNGTQLQNFTLDRSSVLVDGYSPNRNEPLTGNSDLPFWAVILIGLAGLLGVITCLICGVLVTTRRRKKEGEYNVQQQCPGYYQSHLDLEDLQ

SEQ ID NO: 151 - protein, 114 aa, synthetic construct
  REGION 1..114: note = MUC16c114-N1
AFSPLARRVDRVAIYEEFLRMTRNGTQLQNFTLDRSSVLVDGYSPNRNEPLTGNSDLPFWAVILIGLAGLLGLITCLICGVLVTTRRRKKEGEYNVQQQCPGYYQSHLDLEDLQ

SEQ ID NO: 152 - protein, 114 aa, synthetic construct
  REGION 1..114: note = MUC16c114-N2
NFSPLARRVDRVAIYEEFLRMTRAGTQLQNFTLDRSSVLVDGYSPNRNEPLTGNSDLPFWAVILIGLAGLLGLITCLICGVLVTTRRRKKEGEYNVQQQCPGYYQSHLDLEDLQ

SEQ ID NO: 153 - protein, 114 aa, synthetic construct
  REGION 1..114: note = MUC16c114-N12
AFSPLARRVDRVAIYEEFLRMTRAGTQLQNFTLDRSSVLVDGYSPNRNEPLTGNSDLPFWAVILIGLAGLLGLITCLICGVLVTTRRRKKEGEYNVQQQCPGYYQSHLDLEDLQ

SEQ ID NO: 154 - protein, 114 aa, synthetic construct
  REGION 1..114: note = MUC16c114-N123
AFSPLARRVDRVAIYEEFLRMTRAGTQLQAFTLDRSSVLVDGYSPNRNEPLTGNSDLPFWAVILIGLAGLLGLITCLICGVLVTTRRRKKEGEYNVQQQCPGYYQSHLDLEDLQ

SEQ ID NO: 155 - protein, 6 aa, synthetic construct
  REGION 1..6: note = MUC16c344 N-term of first tandem repeat
WELSQL

SEQ ID NO: 156 - protein, 7 aa, synthetic construct
  REGION 1..7: note = MUC16c344 C-term of first tandem repeat
TGVDSLC

SEQ ID NO: 157 - protein, 7 aa, synthetic construct
  REGION 1..7: note = MUC16c344 N-term of ectodomain
NFSPLAR

SEQ ID NO: 158 - protein, 7 aa, synthetic construct
  REGION 1..7: note = MUC16c344 C-term of ectodomain
TGNSDLP

SEQ ID NO: 159 - protein, 25 aa, synthetic construct
  REGION 1..25: note = Transmembrane
FWAVILIGLAGLLGLITCLICGVLV

SEQ ID NO: 160 - protein, 31 aa, synthetic construct
  REGION 1..31: note = Cytoplasmic tail
TTRRRKKEGEYNVQQQCPGYYQSHLDLEDLQ

SEQ ID NO: 161 - protein, 58 aa, synthetic construct
  REGION 1..58: note = MUC16c114 ectodomain
NFSPLARRVDRVAIYEEFLRMTRNGTQLQNFTLDRSSVLVDGYSPNRNEPLTGNSDLP

SEQ ID NO: 162 - protein, 24 aa, synthetic construct
  REGION 1..24: note = MUC16c80 ectodomain
NFSPLARRVDRVAIYEEFLRMDLP

SEQ ID NO: 163 - protein, 58 aa, synthetic construct; identical to SEQ ID NO: 161
  REGION 1..58: note = MUC16c86 ectodomain

SEQ ID NO: 164 - protein, 22 aa, synthetic construct
  REGION 1..22: note = MUC16c86 transmembrane
FWAVILIGLAGLLGLITCLICG

SEQ ID NO: 165 - protein, 6 aa, synthetic construct
  REGION 1..6: note = MUC16c86 cytoplasmic
DLEDLQ

SEQ ID NO: 166 - protein, 58 aa, synthetic construct
  REGION 1..58: note = MUC16 3(N to A)c114 ectodomain
AFSPLARRVDRVAIYEEFLRMTRAGTQLQAFTLDRSSVLVDGYSPNRNEPLTGNSDLP

SEQ ID NO: 167 - protein, 128 aa, synthetic construct
  REGION 1..128: note = LGALS3 sugar binding domain
PYNLPLPGGVVPRMLITILGTVKPNANRIALDFQRGNDVAFHFNPRFNENNRRVIVCNTKLDNNWGREERQSVFPFESGKPFKIQVLVEPDHFKVAVNDAHLLQYNHRVKKLNEISKLGISGDIDLTS

SEQ ID NO: 168 - protein, 19 aa, synthetic construct
  REGION 1..19: note = MUC16 nonglycosylated peptide 2
CTLDRSSVLVDGYSPNRNE

SEQ ID NO: 169 - protein, 18 aa, synthetic construct
  REGION 1..18: note = MUC16 unrelated peptide 18mer
GAVPRSATINVSRIATGP

SEQ ID NO: 170 - protein, 17 aa, synthetic construct
  REGION 1..17: note = 18mer (no C)
TRNGTQLQNFTLDRSSV

SEQ ID NO: 171 - protein, 14 aa, synthetic construct
  REGION 1..14: note = 15mer (no C)
GTQLQNFTLDRSSV

SEQ ID NO: 172 - protein, 114 aa, synthetic construct
  REGION 1..114: note = MUC16c114-N23
NFSPLARRVDRVAIYEEFLRMTRAGTQLQAFTLDRSSVLVDGYSPNRNEPLTGNSDLPFWAVILIGLAGLLGLITCLICGVLVTTRRRKKEGEYNVQQQCPGYYQSHLDLEDLQ

SEQ ID NO: 173 - protein, 344 aa, synthetic construct
  REGION 1..344: note = N24 mut c344
WELSQLTHGVTQLGFYVLDRDSLFINGYAPQNLSIRGEYQINFHIVNQNLSNPDPTSSEYITLLRDIQDKVTTLYKGSQLHDTFRFCLVTNLTMDSVLVTVKALFSSNLDPSLVEQVFLDKTLNASFHQLGSTYQLVDIHVTEMESSVYQPTSSSSTQHFYLNFTITNLPYSQDKAQPGTTNYQRNKRNIEDALNQLFRNSSIKSYFSDCQVSTFRSVPNRHHTGVDSLCNFSPLARRVDRVAIYEEFLRMTRAGTQLQNFTLDRSSVLVDGYSPNRNEPLTGNSDLPFWAVILIGLAGLLGLITCLICGVLVTTRRRKKEGEYNVQQQCPGYYQSHLDLEDLQ

SEQ ID NO: 174 - protein, 344 aa, synthetic construct
  REGION 1..344: note = N30 mut c344
WELSQLTHGVTQLGFYVLDRDSLFINGYAPQNLSIRGEYQINFHIVNQNLSNPDPTSSEYITLLRDIQDKVTTLYKGSQLHDTFRFCLVTNLTMDSVLVTVKALFSSNLDPSLVEQVFLDKTLNASFHQLGSTYQLVDIHVTEMESSVYQPTSSSSTQHFYLNFTITNLPYSQDKAQPGTTNYQRNKRNIEDALNQLFRNSSIKSYFSDCQVSTFRSVPNRHHTGVDSLCNFSPLARRVDRVAIYEEFLRMTRNGTQLQAFTLDRSSVLVDGYSPNRNEPLTGNSDLPFWAVILIGLAGLLGLITCLICGVLVTTRRRKKEGEYNVQQQCPGYYQSHLDLEDLQ

SEQ ID NO: 175 - protein, 344 aa, synthetic construct
  REGION 1..344: note = N24-N30 mut c344
WELSQLTHGVTQLGFYVLDRDSLFINGYAPQNLSIRGEYQINFHIVNQNLSNPDPTSSEYITLLRDIQDKVTTLYKGSQLHDTFRFCLVTNLTMDSVLVTVKALFSSNLDPSLVEQVFLDKTLNASFHQLGSTYQLVDIHVTEMESSVYQPTSSSSTQHFYLNFTITNLPYSQDKAQPGTTNYQRNKRNIEDALNQLFRNSSIKSYFSDCQVSTFRSVPNRHHTGVDSLCNFSPLARRVDRVAIYEEFLRMTRAGTQLQAFTLDRSSVLVDGYSPNRNEPLTGNSDLPFWAVILIGLAGLLGLITCLICGVLVTTRRRKKEGEYNVQQQCPGYYQSHLDLEDLQ